European Patent Specification EP 3 986 428 B1, published May 29, 2024. Title: All-in One vector for CAR and therapeutic effector molecule. Applicant: Medizinische Hochschule Hannover. The sequence listing filed with the application follows.

SEQUENCE LISTING (35 sequences)

SEQ ID NO: 1 - DNA, 244 bp, Artificial Sequence
  NFATenhsyn promoter
  TATA_signal 202..208: /note="TATA box"
tggaggaaaaactgtttcatacagaaggcgtggaggaaaaactgtttcatacagaaggcgtggaggaaaaactgtttcatacagaaggcgtggaggaaaaactgtttcatacagaaggcgtggaggaaaaactgtttcatacagaaggcgtggaggaaaaactgtttcatacagaaggcgtctgcaggagactctagagggtatataatggtttaaacttaagcttggtaccgggcccccgaag

SEQ ID NO: 2 - DNA, 364 bp, Artificial Sequence
  NFATmIL2 promoter
  TATA_signal 291..297: /note="TATA box"
gatatcgaattaggaggaaaaactgtttcatacagaaggcgtcaattaggaggaaaaactgtttcatacagaaggcgtcaattaggaggaaaaactgtttcatacagaaggcgtcaattggtcccatcgaattaggaggaaaaactgtttcatacagaaggcgtcaattaggaggaaaaactgtttcatacagaaggcgtcaattaggaggaaaaactgtttcatacagaaggcgtcaattggtcccgggacattttgacacccccataatatttttccagaattaacagtataaattgcatctcttgttcaagagttccctatcactctctttaatcactactcacagtaacctcaactcctg

SEQ ID NO: 3 - DNA, 173 bp, Artificial Sequence
  NFκBenhsyn promoter
  TATA_signal 131..137: /note="TATA box"
ctcgaggggaatttccggggactttccgggaatttccggggactttccgggaatttccgggaatttccggggactttccgggaatttccggggactttccgggaatttccctgcaggagactctagagggtatataatggtttaaacttaagcttggtaccgggcccccgaag

SEQ ID NO: 4 - DNA, 1623 bp, Artificial Sequence
  IL-12 coding sequence
  CDS 1..1623: /note="synthetic coding sequence for IL-12" /transl_table=1
atgtgtcaccagcagctggtcatcagctggttcagcctggtgttcctggcctctcctctggtggccatctgggagctgaagaaagacgtgtacgtggtggaactggactggtatcccgatgctcctggcgagatggtggtgctgacctgcgatacccctgaagaggacggcatcacctggacactggatcagtctagcgaggtgctcggcagcggcaagaccctgaccatccaagtgaaagagtttggcgacgccggccagtacacctgtcacaaaggcggagaagtgctgagccacagcctgctgctgctccacaagaaagaggatggcatttggagcaccgacatcctgaaggaccagaaagagcccaagaacaagaccttcctgagatgcgaggccaagaactacagcggccggttcacatgttggtggctgaccaccatcagcaccgacctgaccttcagcgtgaagtccagcagaggcagcagtgatcctcagggcgttacatgtggcgccgctacactgtctgccgaaagagtgcggggcgacaacaaagaatacgagtacagcgtggaatgccaagaggacagcgcctgtccagccgccgaagagtctctgcctatcgaagtgatggtggacgccgtgcacaagctgaagtacgagaactacacctccagctttttcatccgggacatcatcaagcccgatcctccaaagaacctgcagctgaagcctctgaagaacagcagacaggtggaagtgtcctgggagtaccccgacacctggtctacaccccacagctacttcagcctgaccttttgcgtgcaagtgcagggcaagtccaagcgcgagaaaaaggaccgggtgttcaccgacaagaccagcgccaccgtgatctgcagaaagaacgccagcatcagcgtcagagcccaggaccgctactacagcagctcttggagcgaatgggccagcgtgccatgttctggtggcggaggatctggcggaggtggaagcggcggaggcggatctagaaatctgcctgtggccactcctgatcctggcatgttcccttgtctgcaccacagccagaacctgctgagagccgtgtccaacatgctgcagaaggccagacagaccctggaattctacccctgcaccagcgaggaaatcgaccacgaggacatcaccaaggataagaccagtaccgtggaagcctgcctgcctctggaactgaccaagaacgagagctgcctgaacagccgggaaaccagcttcatcaccaacggctcttgcctggccagcagaaagacctccttcatgatggccctgtgcctgagcagcatctacgaggacctgaagatgtaccaggtggaattcaagaccatgaacgccaagctgctgatggaccccaagcggcagatcttcctggaccagaatatgctggccgtgatcgacgagctgatgcaggccctgaacttcaacagcgagacagtgccccagaagtctagcctggaagaacccgacttctacaagaccaagatcaagctgtgcatcctgctgcacgccttccgcatcagagccgtgaccatcgatagagtgatgagctacctgaacgcctcctga

SEQ ID NO: 5 - protein, 540 aa, Artificial Sequence
  [CDS]:1..1623 from SEQ ID NO 4
MCHQQLVISWFSLVFLASPLVAIWELKKDVYVVELDWYPDAPGEMVVLTCDTPEEDGITWTLDQSSEVLGSGKTLTIQVKEFGDAGQYTCHKGGEVLSHSLLLLHKKEDGIWSTDILKDQKEPKNKTFLRCEAKNYSGRFTCWWLTTISTDLTFSVKSSRGSSDPQGVTCGAATLSAERVRGDNKEYEYSVECQEDSACPAAEESLPIEVMVDAVHKLKYENYTSSFFIRDIIKPDPPKNLQLKPLKNSRQVEVSWEYPDTWSTPHSYFSLTFCVQVQGKSKREKKDRVFTDKTSATVICRKNASISVRAQDRYYSSSWSEWASVPCSGGGGSGGGGSGGGGSRNLPVATPDPGMFPCLHHSQNLLRAVSNMLQKARQTLEFYPCTSEEIDHEDITKDKTSTVEACLPLELTKNESCLNSRETSFITNGSCLASRKTSFMMALCLSSIYEDLKMYQVEFKTMNAKLLMDPKRQIFLDQNMLAVIDELMQALNFNSETVPQKSSLEEPDFYKTKIKLCILLHAFRIRAVTIDRVMSYLNAS

SEQ ID NO: 6 - DNA, 534 bp, Artificial Sequence
  synthetic coding sequence for IL-18
  CDS 1..534: /note="synthetic coding sequence for IL-18" /transl_table=1
atggcctggaccgttctcctcctcggcctcctctctcactgcacaggctctgtgacctcctactttggcaagcttgaatctaaattatcagtcataagaaatttgaatgaccaagttctcttcattgaccaaggaaatcggcctctatttgaagatatgactgattctgactgtagagataatgcaccccggaccatatttattataagtatgtataaagatagccagcctagaggtatggctgtaactatctctgtgaagtgtgagaaaatttcaactctctcctgtgagaacaaaattatttcctttaaggaaatgaatcctcctgataacatcaaggatacaaaaagtgacatcatattctttcagagaagtgtcccaggacatgataataagatgcaatttgaatcttcatcatacgaaggatactttctagcttgtgaaaaagagagagacctttttaaactcattttgaaaaaagaggatgaattgggggatagatctataatgttcactgttcaaaacgaagactag

SEQ ID NO: 7 - protein, 177 aa, Artificial Sequence
  [CDS]:1..534 from SEQ ID NO 6
MAWTVLLLGLLSHCTGSVTSYFGKLESKLSVIRNLNDQVLFIDQGNRPLFEDMTDSDCRDNAPRTIFIISMYKDSQPRGMAVTISVKCEKISTLSCENKIISFKEMNPPDNIKDTKSDIIFFQRSVPGHDNKMQFESSSYEGYFLACEKERDLFKLILKKEDELGDRSIMFTVQNED

SEQ ID NO: 8 - DNA, 9555 bp, Artificial Sequence
  pCCL.PPT.NFATenhsyn.EGFP.PGK.CAR.wPRE
  promoter 1785..2455: /function="CMV promoter"
  LTR 2456..2636: /note="5´ LTR truncated"
  misc_signal 2683..2808: /note="packaging signal of HIV-1"
  misc_signal 3301..3534: /note="RRE of HIV-1"
  misc_signal 3302..3543: /note="PRE"
  terminator 4027..4150: /note="cPPT/CTScPPT/CTS, central polypurine tract and central termination sequence of HIV-1"
  promoter 4174..4417: /note="NFATenhsyn"
  CDS 4430..5149: /gene="EGFP" /transl_table=1
  promoter 5158..5673: /note="PGK promoter"
  gene 5705..7159: /gene="placeholder for CAR"
  misc_signal 7186..7774: /note="WPRE"
  LTR 7861..8094: /note="3´ LTR (∆ U3)"
agtactcaccagtcacagaaaagcatcttacggatggcatgacagtaagagaattatgcagtgctgccataaccatgagtgataacactgcggccaacttacttctgacaacgatcggaggaccgaaggagctaaccgcttttttgcacaacatgggggatcatgtaactcgccttgatcgttgggaaccggagctgaatgaagccataccaaacgacgagcgtgacaccacgatgcctgtagcaatggcaacaacgttgcgcaaactattaactggcgaactacttactctagcttcccggcaacaattaatagactggatggaggcggataaagttgcaggaccacttctgcgctcggcccttccggctggctggtttattgctgataaatctggagccggtgagcgtgggtctcgcggtatcattgcagcactggggccagatggtaagccctcccgtatcgtagttatctacacgacggggagtcaggcaactatggatgaacgaaatagacagatcgctgagataggtgcctcactgattaagcattggtaactgtcagaccaagtttactcatatatactttagattgatttaaaacttcatttttaatttaaaaggatctaggtgaagatcctttttgataatctcatgaccaaaatcccttaacgtgagttttcgttccactgagcgtcagaccccgtagaaaagatcaaaggatcttcttgagatcctttttttctgcgcgtaatctgctgcttgcaaacaaaaaaaccaccgctaccagcggtggtttgtttgccggatcaagagctaccaactctttttccgaaggtaactggcttcagcagagcgcagataccaaatactgttcttctagtgtagccgtagttaggccaccacttcaagaactctgtagcaccgcctacatacctcgctctgctaatcctgttaccagtggctgctgccagtggcgataagtcgtgtcttaccgggttggactcaagacgatagttaccggataaggcgcagcggtcgggctgaacggggggttcgtgcacacagcccagcttggagcgaacgacctacaccgaactgagatacctacagcgtgagctatgagaaagcgccacgcttcccgaagggagaaaggcggacaggtatccggtaagcggcagggtcggaacaggagagcgcacgagggagcttccagggggaaacgcctggtatctttatagtcctgtcgggtttcgccacctctgacttgagcgtcgatttttgtgatgctcgtcaggggggcggagcctatggaaaaacgccagcaacgcggcctttttacggttcctggccttttgctggccttttgctcacatgttctttcctgcgttatcccctgattctgtggataaccgtattaccgcctttgagtgagctgataccgctcgccgcagccgaacgaccgagcgcagcgagtcagtgagcgaggaagcggaagagcgcccaatacgcaaaccgcctctccccgcgcgttggccgattcattaatgcagctggcacgacaggtttcccgactggaaagcgggcagtgagcgcaacgcaattaatgtgagttagctcactcattaggcaccccaggctttacactttatgcttccggctcgtatgttgtgtggaattgtgagcggataacaatttcacacaggaaacagctatgaccatgattacgccaagcgcgcaattaaccctcactaaagggaacaaaagctggagctgcaagcttggccattgcatacgttgtatccatatcataatatgtacatttatattggctcatgtccaacattaccgccatgttgacattgattattgactagttattaatagtaatcaattacggggtcattagttcatagcccatatatggagttccgcgttacataacttacggtaaatggcccgcctggctgaccgcccaacgacccccgcccattgacgtcaataatgacgtatgttcccatagtaacgccaatagggactttccattgacgtcaatgggtggagtatttacggtaaactgcccacttggcagtacatcaagtgtatcatatgccaagtacgccccctattgacgtcaatgacggtaaatggcccgcctggcattatgcccagtacatgaccttatgggactttcctacttggcagtacatctacgtattagtcatcgctattaccatggtgatgcggttttggcagtacatcaatgggcgtggatagcggtttgactcacggggatttccaagtctccaccccattgacgtcaatgggagtttgttttggcaccaaaatcaacgggactttccaaaatgtcgtaacaactccgccccattgacgcaaatgggcggtaggcgtgtacggtgggaggtctatataagcagagctcgtttagtgaaccggggtctctctggttagaccagatctgagcctgggagctctctggctaactagggaacccactgcttaagcctcaataaagcttgccttgagtgcttcaagtagtgtgtgcccgtctgttgtgtgactctggtaactagagatccctcagacccttttagtcagtgtggaaaatctctagcagtggcgcccgaacagggacttgaaagcgaaagggaaaccagaggagctctctcgacgcaggactcggcttgctgaagcgcgcacggcaagaggcgaggggcggcgactggtgagtacgccaaaaattttgactagcggaggctagaaggagagagatgggtgcgagagcgtcagtattaagcgggggagaattagatcgcgatgggaaaaaattcggttaaggccagggggaaagaaaaaatataaattaaaacatatagtatgggcaagcagggagctagaacgattcgcagttaatcctggcctgttagaaacatcagaaggctgtagacaaatactgggacagctacaaccatcccttcagacaggatcagaagaacttagatcattatataatacagtagcaaccctctattgtgtgcatcaaaggatagagataaaagacaccaaggaagctttagacaagatagaggaagagcaaaacaaaagtaagaccaccgcacagcaagcggccgctgatcttcagacctggaggaggagatatgagggacaattggagaagtgaattatataaatataaagtagtaaaaattgaaccattaggagtagcacccaccaaggcaaagagaagagtggtgcagagagaaaaaagagcagtgggaataggagctttgttccttgggttcttgggagcagcaggaagcactatgggcgcagcctcaatgacgctgacggtacaggccagacaattattgtctggtatagtgcagcagcagaacaatttgctgagggctattgaggcgcaacagcatctgttgcaactcacagtctggggcatcaagcagctccaggcaagaatcctggctgtggaaagatacctaaaggatcaacagctcctggggatttggggttgctctggaaaactcatttgcaccactgctgtgccttggaatgctagttggagtaataaatctctggaacagatttggaatcacacgacctggatggagtgggacagagaaattaacaattacacaagcttaatacactccttaattgaagaatcgcaaaaccagcaagaaaagaatgaacaagaattattggaattagataaatgggcaagtttgtggaattggtttaacataacaaattggctgtggtatataaaattattcataatgatagtaggaggcttggtaggtttaagaatagtttttgctgtactttctatagtgaatagagttaggcagggatattcaccattatcgtttcagacccacctcccaaccccgaggggacccgacaggcccgaaggaatagaagaagaaggtggagagagagacagagacagatccattcgattagtgaacggatctcgacggtatcggttaacttttaaaagaaaaggggggattggggggtacagtgcaggggaaagaatagtagacataatagcaacagacatacaaactaaagaattacaaaaacaaattacaaaaattcaaaattttatcgatcacgagactagcctcgagcgtggaggaaaaactgtttcatacagaaggcgtggaggaaaaactgtttcatacagaaggcgtggaggaaaaactgtttcatacagaaggcgtggaggaaaaactgtttcatacagaaggcgtggaggaaaaactgtttcatacagaaggcgtggaggaaaaactgtttcatacagaaggcgtctgcaggagactctagagggtatataatggtttaaacttaagcttggtaccgggcccccgaagacgcgtgccaccatggtgagcaagggcgaggagctgttcaccggggtggtgcccatcctggtcgagctggacggcgacgtaaacggccacaagttcagcgtgtccggcgagggcgagggcgatgccacctacggcaagctgaccctgaagttcatctgcaccaccggcaagctgcccgtgccctggcccaccctcgtgaccaccctgacctacggcgtgcagtgcttcagccgctaccccgaccacatgaagcagcacgacttcttcaagtccgccatgcccgaaggctacgtccaggagcgcaccatcttcttcaaggacgacggcaactacaagacccgcgccgaggtgaagttcgagggcgacaccctggtgaaccgcatcgagctgaagggcatcgacttcaaggaggacggcaacatcctggggcacaagctggagtacaactacaacagccacaacgtctatatcatggccgacaagcagaagaacggcatcaaggtgaacttcaagatccgccacaacatcgaggacggcagcgtgcagctcgccgaccactaccagcagaacacccccatcggcgacggccccgtgctgctgcccgacaaccactacctgagcacccagtccgccctgagcaaagaccccaacgagaagcgcgatcacatggtcctgctggagttcgtgaccgccgccgggatcactctcggcatggacgagctgtacaagtaatcgaattcccacggggttggggttgcgccttttccaaggcagccctgggtttgcgcagggacgcggctgctctgggcgtggttccgggaaacgcagcggcgccgaccctgggtctcgcacattcttcacgtccgttcgcagcgtcacccggatcttcgccgctacccttgtgggccccccggcgacgcttcctgctccgcccctaagtcgggaaggttccttgcggttcgcggcgtgccggacgtgacaaacggaagccgcacgtctcactagtaccctcgcagacggacagcgccagggagcaatggcagcgcgccgaccgcgatgggctgtggccaatagcggctgctcagcggggcgcgccgagagcagcggccgggaaggggcggtgcgggaggcggggtgtggggcggtagtgtgggccctgttcctgcccgcgcggtgttccgcattctgcaagcctccggagcgcacgtcggcagtcggctccctcgttgaccgaatcaccgacctctctccccagggggatccaccggtcacgtggctagcgccaccnnnnnnnnnnnnnnnnnnnnnnnnnnnnnnnnnnnnnnnnnnnnnnnnnnnnnnnnnnnnnnnnnnnnnnnnnnnnnnnnnnnnnnnnnnnnnnnnnnnnnnnnnnnnnnnnnnnnnnnnnnnnnnnnnnnnnnnnnnnnnnnnnnnnnnnnnnnnnnnnnnnnnnnnnnnnnnnnnnnnnnnnnnnnnnnnnnnnnnnnnnnnnnnnnnnnnnnnnnnnnnnnnnnnnnnnnnnnnnnnnnnnnnnnnnnnnnnnnnnnnnnnnnnnnnnnnnnnnnnnnnnnnnnnnnnnnnnnnnnnnnnnnnnnnnnnnnnnnnnnnnnnnnnnnnnnnnnnnnnnnnnnnnnnnnnnnnnnnnnnnnnnnnnnnnnnnnnnnnnnnnnnnnnnnnnnnnnnnnnnnnnnnnnnnnnnnnnnnnnnnnnnnnnnnnnnnnnnnnnnnnnnnnnnnnnnnnnnnnnnnnnnnnnnnnnnnnnnnnnnnnnnnnnnnnnnnnnnnnnnnnnnnnnnnnnnnnnnnnnnnnnnnnnnnnnnnnnnnnnnnnnnnnnnnnnnnnnnnnnnnnnnnnnnnnnnnnnnnnnnnnnnnnnnnnnnnnnnnnnnnnnnnnnnnnnnnnnnnnnnnnnnnnnnnnnnnnnnnnnnnnnnnnnnnnnnnnnnnnnnnnnnnnnnnnnnnnnnnnnnnnnnnnnnnnnnnnnnnnnnnnnnnnnnnnnnnnnnnnnnnnnnnnnnnnnnnnnnnnnnnnnnnnnnnnnnnnnnnnnnnnnnnnnnnnnnnnnnnnnnnnnnnnnnnnnnnnnnnnnnnnnnnnnnnnnnnnnnnnnnnnnnnnnnnnnnnnnnnnnnnnnnnnnnnnnnnnnnnnnnnnnnnnnnnnnnnnnnnnnnnnnnnnnnnnnnnnnnnnnnnnnnnnnnnnnnnnnnnnnnnnnnnnnnnnnnnnnnnnnnnnnnnnnnnnnnnnnnnnnnnnnnnnnnnnnnnnnnnnnnnnnnnnnnnnnnnnnnnnnnnnnnnnnnnnnnnnnnnnnnnnnnnnnnnnnnnnnnnnnnnnnnnnnnnnnnnnnnnnnnnnnnnnnnnnnnnnnnnnnnnnnnnnnnnnnnnnnnnnnnnnnnnnnnnnnnnnnnnnnnnnnnnnnnnnnnnnnnnnnnnnnnnnnnnnnnnnnnnnnnnnnnnnnnnnnnnnnnnnnnnnnnnnnnnnnnnnnnnnnnnnnnnnnnnnnnnnnnnnnnnnnnnnnnnnnnnnnnnnnnnnnnnnnnnnnnnnnnnnnnnnnnnnnnnnnnnnnnnnnnnnnnnnnnnnnnnnnnnnnnnnnnnnnnnnnnnnnnnnnnnnnnnnnnnnnnnnnnnnnnnnnnnnnnnnnnnnnnnnnnnnnnnnnnnnnnnnnnnnnnnnnnnnnnnnnnnnnnnnnnnnnnnnnnnnnnnnnnnnnnnnnnnnnnnnnnnnnnnnnnnnnnnnnnnnnnnnntaggatccgccggcggccgcgtcgacaatcaacctctggattacaaaatttgtgaaagattgactggtattcttaactatgttgctccttttacgctatgtggatacgctgctttaatgcctttgtatcatgctattgcttcccgtatggctttcattttctcctccttgtataaatcctggttgctgtctctttatgaggagttgtggcccgttgtcaggcaacgtggcgtggtgtgcactgtgtttgctgacgcaacccccactggttggggcattgccaccacctgtcagctcctttccgggactttcgctttccccctccctattgccacggcggaactcatcgccgcctgccttgcccgctgctggacaggggctcggctgttgggcactgacaattccgtggtgttgtcggggaagctgacgtcctttccatggctgctcgcctgtgttgccacctggattctgcgcgggacgtccttctgctacgtcccttcggccctcaatccagcggaccttccttcccgcggcctgctgccggctctgcggcctcttccgcgtcttcgccttcgccctcagacgagtcggatctccctttgggccgcctccccgcctggaattcgagctcggtacctttaagaccaatgacttacaaggcagctgtagatcttagccactttttaaaagaaaaggggggactggaagggctaattcactcccaacgaagacaagatctgctttttgcttgtactgggtctctctggttagaccagatctgagcctgggagctctctggctaactagggaacccactgcttaagcctcaataaagcttgccttgagtgcttcaagtagtgtgtgcccgtctgttgtgtgactctggtaactagagatccctcagacccttttagtcagtgtggaaaatctctagcagtagtagttcatgtcatcttattattcagtatttataacttgcaaagaaatgaatatcagagagtgagaggaacttgtttattgcagcttataatggttacaaataaagcaatagcatcacaaatttcacaaataaagcatttttttcactgcattctagttgtggtttgtccaaactcatcaatgtatcttatcatgtctggctctagctatcccgcccctaactccgcccagttccgcccattctccgccccatggctgactaattttttttatttatgcagaggccgaggccgcctcggcctctgagctattccagaagtagtgaggaggcttttttggaggcctaggcttttgcgtcgagacgtacccaattcgccctatagtgagtcgtattacgcgcgctcactggccgtcgttttacaacgtcgtgactgggaaaaccctggcgttacccaacttaatcgccttgcagcacatccccctttcgccagctggcgtaatagcgaagaggcccgcaccgatcgcccttcccaacagttgcgcagcctgaatggcgaatggcgcgacgcgccctgtagcggcgcattaagcgcggcgggtgtggtggttacgcgcagcgtgaccgctacacttgccagcgccctagcgcccgctcctttcgctttcttcccttcctttctcgccacgttcgccggctttccccgtcaagctctaaatcgggggctccctttagggttccgatttagtgctttacggcacctcgaccccaaaaaacttgattagggtgatggttcacgtagtgggccatcgccctgatagacggtttttcgccctttgacgttggagtccacgttctttaatagtggactcttgttccaaactggaacaacactcaaccctatctcggtctattcttttgatttataagggattttgccgatttcggcctattggttaaaaaatgagctgatttaacaaaaatttaacgcgaattttaacaaaatattaacgtttacaatttcccaggtggcacttttcggggaaatgtgcgcggaacccctatttgtttatttttctaaatacattcaaatatgtatccgctcatgagacaataaccctgataaatgcttcaataatattgaaaaaggaagagtatgagtattcaacatttccgtgtcgcccttattcccttttttgcggcattttgccttcctgtttttgctcacccagaaacgctggtgaaagtaaaagatgctgaagatcagttgggtgcacgagtgggttacatcgaactggatctcaacagcggtaagatccttgagagttttcgccccgaagaacgttttccaatgatgagcacttttaaagttctgctatgtggcgcggtattatcccgtattgacgccgggcaagagcaactcggtcgccgcatacactattctcagaatgacttggttg

SEQ ID NO: 9 - protein, 239 aa, Artificial Sequence
  [CDS]:4430..5149 from SEQ ID NO 8
MVSKGEELFTGVVPILVELDGDVNGHKFSVSGEGEGDATYGKLTLKFICTTGKLPVPWPTLVTTLTYGVQCFSRYPDHMKQHDFFKSAMPEGYVQERTIFFKDDGNYKTRAEVKFEGDTLVNRIELKGIDFKEDGNILGHKLEYNYNSHNVYIMADKQKNGIKVNFKIRHNIEDGSVQLADHYQQNTPIGDGPVLLPDNHYLSTQSALSKDPNEKRDHMVLLEFVTAAGITLGMDELYK

SEQ ID NO: 10 - DNA, 407 bp, Artificial Sequence
  SFFV promoter
gtaacgccattttgcaaggcatggaaaaataccaaaccaagaatagagaagttcagatcaagggcgggtacatgaaaatagctaacgttgggccaaacaggatatctgcggtgagcagtttcggccccggcccggggccaagaacagatggtcaccgcagtttcggccccggcccgaggccaagaacagatggtccccagatatggcccaaccctcagcagtttcttaagacccatcagatgtttccaggctcccccaaggacctgaaatgaccctgcgccttatttgaattaaccaatcagcctgcttctcgcttctgttcgcgcgcttctgcttcccgagctctataaaagagctcacaacccctcactcggcgcgccagtcctccgacagactgagtcggccgg

SEQ ID NO: 11 - DNA, 245 bp, Artificial Sequence
  EF-1 alpha promoter
tggctccggtgcccgtcagtgggcagagcgcacatcgcccacagtccccgagaagttggggggaggggtcggcaattgaaccggtgcctagagaaggtggcgcggggtaaactgggaaagtgatgtcgtgtactggctccgcctttttcccgagggtgggggagaaccgtatataagtgcagtagtcgccgtgaacgttctttttcgcaacgggtttgccgccagaacacaggtgtcgtgacgcg

SEQ ID NO: 12 - DNA, 671 bp, Artificial Sequence
  CMV promoter element
ccattgcatacgttgtatccatatcataatatgtacatttatattggctcatgtccaacattaccgccatgttgacattgattattgactagttattaatagtaatcaattacggggtcattagttcatagcccatatatggagttccgcgttacataacttacggtaaatggcccgcctggctgaccgcccaacgacccccgcccattgacgtcaataatgacgtatgttcccatagtaacgccaatagggactttccattgacgtcaatgggtggagtatttacggtaaactgcccacttggcagtacatcaagtgtatcatatgccaagtacgccccctattgacgtcaatgacggtaaatggcccgcctggcattatgcccagtacatgaccttatgggactttcctacttggcagtacatctacgtattagtcatcgctattaccatggtgatgcggttttggcagtacatcaatgggcgtggatagcggtttgactcacggggatttccaagtctccaccccattgacgtcaatgggagtttgttttggcaccaaaatcaacgggactttccaaaatgtcgtaacaactccgccccattgacgcaaatgggcggtaggcgtgtacggtgggaggtctatataagcagagctcgtttagtgaaccg

SEQ ID NO: 13 - DNA, 232 bp, Artificial Sequence
  RSV promoter element
ttaatgtagtcttatgcaatactcttgtagtcttgcaacatggtaacgatgagttagcaacatgccttacaaggagagaaaaagcaccgtgcatgccgattggtggaagtaaggtggtacgatcgtgccttattaggaaggcaacagacgggtctgacatggattggacgaaccactgaattgccgcattgcagagatattgtatttaagtgcctagctcgatacaataaac

SEQ ID NO: 14 - DNA, 454 bp, Artificial Sequence
  HIV U3 promoter element
ttggaagggctaattcactcccaaagaagacaagatatccttgatctgtggatctaccacacacaaggctacttccctgattagcagaactacacaccagggccaggggtcagatatccactgacctttggatggtgctacaagctagtaccagttgagccagataaggtagaagaggccaataaaggagagaacaccagcttgttacaccctgtgagcctgcatgggatggatgacccggagagagaagtgttagagtggaggtttgacagccgcctagcatttcatcacgtggcccgagagctgcatccggagtacttcaagaactgctgatatcgagcttgctacaagggactttccgctggggactttccagggaggcgtggcctgggcgggactggggagtggcgagccctcagatcctgcatataagcagctgctttttgcctgtact

SEQ ID NO: 15 - DNA, 589 bp, Artificial Sequence
  WPRE element
aatcaacctctggattacaaaatttgtgaaagattgactggtattcttaactatgttgctccttttacgctatgtggatacgctgctttaatgcctttgtatcatgctattgcttcccgtatggctttcattttctcctccttgtataaatcctggttgctgtctctttatgaggagttgtggcccgttgtcaggcaacgtggcgtggtgtgcactgtgtttgctgacgcaacccccactggttggggcattgccaccacctgtcagctcctttccgggactttcgctttccccctccctattgccacggcggaactcatcgccgcctgccttgcccgctgctggacaggggctcggctgttgggcactgacaattccgtggtgttgtcggggaagctgacgtcctttccatggctgctcgcctgtgttgccacctggattctgcgcgggacgtccttctgctacgtcccttcggccctcaatccagcggaccttccttcccgcggcctgctgccggctctgcggcctcttccgcgtcttcgccttcgccctcagacgagtcggatctccctttgggccgcctccccgc

SEQ ID NO: 16 - DNA, 10469 bp, Artificial Sequence
  pCCL.PPT.NFATenhsyn.humanIL12.PGK.CAR.wPRE
  promoter 1785..2455: /note="CMV promoter"
  LTR 2456..2636: /note="5´ LTR truncated"
  misc_signal 2683..2808: /note="packaging signal of HIV-1"
  misc_signal 3301..3534: /note="RRE: rev response element of HIV-1"
  misc_signal 3302..3543: /note="PRE of HIV-1"
  terminator 4027..4150: /note="cPPT/CTScPPT/CTS: central polypurine tract and central termination sequence of HIV-1"
  promoter 4174..4417: /note="NFATenhsyn"
  CDS 4430..6052: /gene="sc IL2 humanized codon usage" /transl_table=1
  promoter 6072..6587: /note="PGK promoter"
  gene 6619..8073: /gene="placeholder for CAR"
  LTR 7861..8094: /note="3´ LTR (∆U3)"
  misc_signal 8100..8688: /note="WPRE"
agtactcaccagtcacagaaaagcatcttacggatggcatgacagtaagagaattatgcagtgctgccataaccatgagtgataacactgcggccaacttacttctgacaacgatcggaggaccgaaggagctaaccgcttttttgcacaacatgggggatcatgtaactcgccttgatcgttgggaaccggagctgaatgaagccataccaaacgacgagcgtgacaccacgatgcctgtagcaatggcaacaacgttgcgcaaactattaactggcgaactacttactctagcttcccggcaacaattaatagactggatggaggcggataaagttgcaggaccacttctgcgctcggcccttccggctggctggtttattgctgataaatctggagccggtgagcgtgggtctcgcggtatcattgcagcactggggccagatggtaagccctcccgtatcgtagttatctacacgacggggagtcaggcaactatggatgaacgaaatagacagatcgctgagataggtgcctcactgattaagcattggtaactgtcagaccaagtttactcatatatactttagattgatttaaaacttcatttttaatttaaaaggatctaggtgaagatcctttttgataatctcatgaccaaaatcccttaacgtgagttttcgttccactgagcgtcagaccccgtagaaaagatcaaaggatcttcttgagatcctttttttctgcgcgtaatctgctgcttgcaaacaaaaaaaccaccgctaccagcggtggtttgtttgccggatcaagagctaccaactctttttccgaaggtaactggcttcagcagagcgcagataccaaatactgttcttctagtgtagccgtagttaggccaccacttcaagaactctgtagcaccgcctacatacctcgctctgctaatcctgttaccagtggctgctgccagtggcgataagtcgtgtcttaccgggttggactcaagacgatagttaccggataaggcgcagcggtcgggctgaacggggggttcgtgcacacagcccagcttggagcgaacgacctacaccgaactgagatacctacagcgtgagctatgagaaagcgccacgcttcccgaagggagaaaggcggacaggtatccggtaagcggcagggtcggaacaggagagcgcacgagggagcttccagggggaaacgcctggtatctttatagtcctgtcgggtttcgccacctctgacttgagcgtcgatttttgtgatgctcgtcaggggggcggagcctatggaaaaacgccagcaacgcggcctttttacggttcctggccttttgctggccttttgctcacatgttctttcctgcgttatcccctgattctgtggataaccgtattaccgcctttgagtgagctgataccgctcgccgcagccgaacgaccgagcgcagcgagtcagtgagcgaggaagcggaagagcgcccaatacgcaaaccgcctctccccgcgcgttggccgattcattaatgcagctggcacgacaggtttcccgactggaaagcgggcagtgagcgcaacgcaattaatgtgagttagctcactcattaggcaccccaggctttacactttatgcttccggctcgtatgttgtgtggaattgtgagcggataacaatttcacacaggaaacagctatgaccatgattacgccaagcgcgcaattaaccctcactaaagggaacaaaagctggagctgcaagcttggccattgcatacgttgtatccatatcataatatgtacatttatattggctcatgtccaacattaccgccatgttgacattgattattgactagttattaatagtaatcaattacggggtcattagttcatagcccatatatggagttccgcgttacataacttacggtaaatggcccgcctggctgaccgcccaacgacccccgcccattgacgtcaataatgacgtatgttcccatagtaacgccaatagggactttccattgacgtcaatgggtggagtatttacggtaaactgcccacttggcagtacatcaagtgtatcatatgccaagtacgccccctattgacgtcaatgacggtaaatggcccgcctggcattatgcccagtacatgaccttatgggactttcctacttggcagtacatctacgtattagtcatcgctattaccatggtgatgcggttttggcagtacatcaatgggcgtggatagcggtttgactcacggggatttccaagtctccaccccattgacgtcaatgggagtttgttttggcaccaaaatcaacgggactttccaaaatgtcgtaacaactccgccccattgacgcaaatgggcggtaggcgtgtacggtgggaggtctatataagcagagctcgtttagtgaaccggggtctctctggttagaccagatctgagcctgggagctctctggctaactagggaacccactgcttaagcctcaataaagcttgccttgagtgcttcaagtagtgtgtgcccgtctgttgtgtgactctggtaactagagatccctcagacccttttagtcagtgtggaaaatctctagcagtggcgcccgaacagggacttgaaagcgaaagggaaaccagaggagctctctcgacgcaggactcggcttgctgaagcgcgcacggcaagaggcgaggggcggcgactggtgagtacgccaaaaattttgactagcggaggctagaaggagagagatgggtgcgagagcgtcagtattaagcgggggagaattagatcgcgatgggaaaaaattcggttaaggccagggggaaagaaaaaatataaattaaaacatatagtatgggcaagcagggagctagaacgattcgcagttaatcctggcctgttagaaacatcagaaggctgtagacaaatactgggacagctacaaccatcccttcagacaggatcagaagaacttagatcattatataatacagtagcaaccctctattgtgtgcatcaaaggatagagataaaagacaccaaggaagctttagacaagatagaggaagagcaaaacaaaagtaagaccaccgcacagcaagcggccgctgatcttcagacctggaggaggagatatgagggacaattggagaagtgaattatataaatataaagtagtaaaaattgaaccattaggagtagcacccaccaaggcaaagagaagagtggtgcagagagaaaaaagagcagtgggaataggagctttgttccttgggttcttgggagcagcaggaagcactatgggcgcagcctcaatgacgctgacggtacaggccagacaattattgtctggtatagtgcagcagcagaacaatttgctgagggctattgaggcgcaacagcatctgttgcaactcacagtctggggcatcaagcagctccaggcaagaatcctggctgtggaaagatacctaaaggatcaacagctcctggggatttggggttgctctggaaaactcatttgcaccactgctgtgccttggaatgctagttggagtaataaatctctggaacagatttggaatcacacgacctggatggagtgggacagagaaattaacaattacacaagcttaatacactccttaattgaagaatcgcaaaaccagcaagaaaagaatgaacaagaattattggaattagataaatgggcaagtttgtggaattggtttaacataacaaattggctgtggtatataaaattattcataatgatagtaggaggcttggtaggtttaagaatagtttttgctgtactttctatagtgaatagagttaggcagggatattcaccattatcgtttcagacccacctcccaaccccgaggggacccgacaggcccgaaggaatagaagaagaaggtggagagagagacagagacagatccattcgattagtgaacggatctcgacggtatcggttaacttttaaaagaaaaggggggattggggggtacagtgcaggggaaagaatagtagacataatagcaacagacatacaaactaaagaattacaaaaacaaattacaaaaattcaaaattttatcgatcacgagactagcctcgagcgtggaggaaaaactgtttcatacagaaggcgtggaggaaaaactgtttcatacagaaggcgtggaggaaaaactgtttcatacagaaggcgtggaggaaaaactgtttcatacagaaggcgtggaggaaaaactgtttcatacagaaggcgtggaggaaaaactgtttcatacagaaggcgtctgcaggagactctagagggtatataatggtttaaacttaagcttggtaccgggcccccgaagacgcgtgccaccatgtgtcaccagcagctggtcatcagctggttcagcctggtgttcctggcctctcctctggtggccatctgggagctgaagaaagacgtgtacgtggtggaactggactggtatcccgatgctcctggcgagatggtggtgctgacctgcgatacccctgaagaggacggcatcacctggacactggatcagtctagcgaggtgctcggcagcggcaagaccctgaccatccaagtgaaagagtttggcgacgccggccagtacacctgtcacaaaggcggagaagtgctgagccacagcctgctgctgctccacaagaaagaggatggcatttggagcaccgacatcctgaaggaccagaaagagcccaagaacaagaccttcctgagatgcgaggccaagaactacagcggccggttcacatgttggtggctgaccaccatcagcaccgacctgaccttcagcgtgaagtccagcagaggcagcagtgatcctcagggcgttacatgtggcgccgctacactgtctgccgaaagagtgcggggcgacaacaaagaatacgagtacagcgtggaatgccaagaggacagcgcctgtccagccgccgaagagtctctgcctatcgaagtgatggtggacgccgtgcacaagctgaagtacgagaactacacctccagctttttcatccgggacatcatcaagcccgatcctccaaagaacctgcagctgaagcctctgaagaacagcagacaggtggaagtgtcctgggagtaccccgacacctggtctacaccccacagctacttcagcctgaccttttgcgtgcaagtgcagggcaagtccaagcgcgagaaaaaggaccgggtgttcaccgacaagaccagcgccaccgtgatctgcagaaagaacgccagcatcagcgtcagagcccaggaccgctactacagcagctcttggagcgaatgggccagcgtgccatgttctggtggcggaggatctggcggaggtggaagcggcggaggcggatctagaaatctgcctgtggccactcctgatcctggcatgttcccttgtctgcaccacagccagaacctgctgagagccgtgtccaacatgctgcagaaggccagacagaccctggaattctacccctgcaccagcgaggaaatcgaccacgaggacatcaccaaggataagaccagtaccgtggaagcctgcctgcctctggaactgaccaagaacgagagctgcctgaacagccgggaaaccagcttcatcaccaacggctcttgcctggccagcagaaagacctccttcatgatggccctgtgcctgagcagcatctacgaggacctgaagatgtaccaggtggaattcaagaccatgaacgccaagctgctgatggaccccaagcggcagatcttcctggaccagaatatgctggccgtgatcgacgagctgatgcaggccctgaacttcaacagcgagacagtgccccagaagtctagcctggaagaacccgacttctacaagaccaagatcaagctgtgcatcctgctgcacgccttccgcatcagagccgtgaccatcgatagagtgatgagctacctgaacgcctcctgatgtacaagtaatcgaattcccacggggttggggttgcgccttttccaaggcagccctgggtttgcgcagggacgcggctgctctgggcgtggttccgggaaacgcagcggcgccgaccctgggtctcgcacattcttcacgtccgttcgcagcgtcacccggatcttcgccgctacccttgtgggccccccggcgacgcttcctgctccgcccctaagtcgggaaggttccttgcggttcgcggcgtgccggacgtgacaaacggaagccgcacgtctcactagtaccctcgcagacggacagcgccagggagcaatggcagcgcgccgaccgcgatgggctgtggccaatagcggctgctcagcggggcgcgccgagagcagcggccgggaaggggcggtgcgggaggcggggtgtggggcggtagtgtgggccctgttcctgcccgcgcggtgttccgcattctgcaagcctccggagcgcacgtcggcagtcggctccctcgttgaccgaatcaccgacctctctccccagggggatccaccggtcacgtggctagcgccaccnnnnnnnnnnnnnnnnnnnnnnnnnnnnnnnnnnnnnnnnnnnnnnnnnnnnnnnnnnnnnnnnnnnnnnnnnnnnnnnnnnnnnnnnnnnnnnnnnnnnnnnnnnnnnnnnnnnnnnnnnnnnnnnnnnnnnnnnnnnnnnnnnnnnnnnnnnnnnnnnnnnnnnnnnnnnnnnnnnnnnnnnnnnnnnnnnnnnnnnnnnnnnnnnnnnnnnnnnnnnnnnnnnnnnnnnnnnnnnnnnnnnnnnnnnnnnnnnnnnnnnnnnnnnnnnnnnnnnnnnnnnnnnnnnnnnnnnnnnnnnnnnnnnnnnnnnnnnnnnnnnnnnnnnnnnnnnnnnnnnnnnnnnnnnnnnnnnnnnnnnnnnnnnnnnnnnnnnnnnnnnnnnnnnnnnnnnnnnnnnnnnnnnnnnnnnnnnnnnnnnnnnnnnnnnnnnnnnnnnnnnnnnnnnnnnnnnnnnnnnnnnnnnnnnnnnnnnnnnnnnnnnnnnnnnnnnnnnnnnnnnnnnnnnnnnnnnnnnnnnnnnnnnnnnnnnnnnnnnnnnnnnnnnnnnnnnnnnnnnnnnnnnnnnnnnnnnnnnnnnnnnnnnnnnnnnnnnnnnnnnnnnnnnnnnnnnnnnnnnnnnnnnnnnnnnnnnnnnnnnnnnnnnnnnnnnnnnnnnnnnnnnnnnnnnnnnnnnnnnnnnnnnnnnnnnnnnnnnnnnnnnnnnnnnnnnnnnnnnnnnnnnnnnnnnnnnnnnnnnnnnnnnnnnnnnnnnnnnnnnnnnnnnnnnnnnnnnnnnnnnnnnnnnnnnnnnnnnnnnnnnnnnnnnnnnnnnnnnnnnnnnnnnnnnnnnnnnnnnnnnnnnnnnnnnnnnnnnnnnnnnnnnnnnnnnnnnnnnnnnnnnnnnnnnnnnnnnnnnnnnnnnnnnnnnnnnnnnnnnnnnnnnnnnnnnnnnnnnnnnnnnnnnnnnnnnnnnnnnnnnnnnnnnnnnnnnnnnnnnnnnnnnnnnnnnnnnnnnnnnnnnnnnnnnnnnnnnnnnnnnnnnnnnnnnnnnnnnnnnnnnnnnnnnnnnnnnnnnnnnnnnnnnnnnnnnnnnnnnnnnnnnnnnnnnnnnnnnnnnnnnnnnnnnnnnnnnnnnnnnnnnnnnnnnnnnnnnnnnnnnnnnnnnnnnnnnnnnnnnnnnnnnnnnnnnnnnnnnnnnnnnnnnnnnnnnnnnnnnnnnnnnnnnnnnnnnnnnnnnnnnnnnnnnnnnnnnnnnnnnnnnnnnnnnnnnnnnnnnnnnnnnnnnnnnnnnnnnnnnnnnnnnnnnnnnnnnnnnnnnnnnnnnnnnnnnnnnnnnnnnnnnnnnnnnnnnnnnnnnnnnnnnnnnnnnnnnnnnnnnnnnnnnnnnnnnnnnnnnnnnnnnnnnnnnnnnnnnnnnnnnnnnnnnnnnnnnnnnnnnnnnnnnnnnnnnnnnnnnnnnnnnnnnnnnnnnnntaggatccgccggcggccgcgtcgacaatcaacctctggattacaaaatttgtgaaagattgactggtattcttaactatgttgctccttttacgctatgtggatacgctgctttaatgcctttgtatcatgctattgcttcccgtatggctttcattttctcctccttgtataaatcctggttgctgtctctttatgaggagttgtggcccgttgtcaggcaacgtggcgtggtgtgcactgtgtttgctgacgcaacccccactggttggggcattgccaccacctgtcagctcctttccgggactttcgctttccccctccctattgccacggcggaactcatcgccgcctgccttgcccgctgctggacaggggctcggctgttgggcactgacaattccgtggtgttgtcggggaagctgacgtcctttccatggctgctcgcctgtgttgccacctggattctgcgcgggacgtccttctgctacgtcccttcggccctcaatccagcggaccttccttcccgcggcctgctgccggctctgcggcctcttccgcgtcttcgccttcgccctcagacgagtcggatctccctttgggccgcctccccgcctggaattcgagctcggtacctttaagaccaatgacttacaaggcagctgtagatcttagccactttttaaaagaaaaggggggactggaagggctaattcactcccaacgaagacaagatctgctttttgcttgtactgggtctctctggttagaccagatctgagcctgggagctctctggctaactagggaacccactgcttaagcctcaataaagcttgccttgagtgcttcaagtagtgtgtgcccgtctgttgtgtgactctggtaactagagatccctcagacccttttagtcagtgtggaaaatctctagcagtagtagttcatgtcatcttattattcagtatttataacttgcaaagaaatgaatatcagagagtgagaggaacttgtttattgcagcttataatggttacaaataaagcaatagcatcacaaatttcacaaataaagcatttttttcactgcattctagttgtggtttgtccaaactcatcaatgtatcttatcatgtctggctctagctatcccgcccctaactccgcccagttccgcccattctccgccccatggctgactaattttttttatttatgcagaggccgaggccgcctcggcctctgagctattccagaagtagtgaggaggcttttttggaggcctaggcttttgcgtcgagacgtacccaattcgccctatagtgagtcgtattacgcgcgctcactggccgtcgttttacaacgtcgtgactgggaaaaccctggcgttacccaacttaatcgccttgcagcacatccccctttcgccagctggcgtaatagcgaagaggcccgcaccgatcgcccttcccaacagttgcgcagcctgaatggcgaatggcgcgacgcgccctgtagcggcgcattaagcgcggcgggtgtggtggttacgcgcagcgtgaccgctacacttgccagcgccctagcgcccgctcctttcgctttcttcccttcctttctcgccacgttcgccggctttccccgtcaagctctaaatcgggggctccctttagggttccgatttagtgctttacggcacctcgaccccaaaaaacttgattagggtgatggttcacgtagtgggccatcgccctgatagacggtttttcgccctttgacgttggagtccacgttctttaatagtggactcttgttccaaactggaacaacactcaaccctatctcggtctattcttttgatttataagggattttgccgatttcggcctattggttaaaaaatgagctgatttaacaaaaatttaacgcgaattttaacaaaatattaacgtttacaatttcccaggtggcacttttcggggaaatgtgcgcggaacccctatttgtttatttttctaaatacattcaaatatgtatccgctcatgagacaataaccctgataaatgcttcaataatattgaaaaaggaagagtatgagtattcaacatttccgtgtcgcccttattcccttttttgcggcattttgccttcctgtttttgctcacccagaaacgctggtgaaagtaaaagatgctgaagatcagttgggtgcacgagtgggttacatcgaactggatctcaacagcggtaagatccttgagagttttcgccccgaagaacgttttccaatgatgagcacttttaaagttctgctatgtggcgcggtattatcccgtattgacgccgggcaagagcaactcggtcgccgcatacactattctcagaatgacttggttg

SEQ ID NO: 17 - protein, 540 aa, Artificial Sequence; identical to SEQ ID NO: 5
  [CDS]:4430..6052 from SEQ ID NO 16

SEQ ID NO: 18 - DNA, 9380 bp, Artificial Sequence
  pCCL.PPT.NFATenhsyn.humanIL18.PGK.CAR.wPRE
  promoter 1785..2455: /note="CMV promoter"
  LTR 2456..2636: /note="5´ LTR truncated"
  misc_signal 2683..2808: /note="packaging signal of HIV-1"
  misc_signal 3301..3534: /note="RRE: rev response element of HIV-1"
  terminator 4030..4147: /note="cPPT/CTS, central polypurine tract and central termination sequence of HIV-1"
  promoter 4174..4417: /note="NFATenhsyn"
  CDS 4430..4963: /gene="signal peptide and human IL18" /transl_table=1
  gene 5530..6984: /note="placeholder for CAR"
  misc_signal 7011..7599: /note="WPRE"
agtactcaccagtcacagaaaagcatcttacggatggcatgacagtaagagaattatgcagtgctgccataaccatgagtgataacactgcggccaacttacttctgacaacgatcggaggaccgaaggagctaaccgcttttttgcacaacatgggggatcatgtaactcgccttgatcgttgggaaccggagctgaatgaagccataccaaacgacgagcgtgacaccacgatgcctgtagcaatggcaacaacgttgcgcaaactattaactggcgaactacttactctagcttcccggcaacaattaatagactggatggaggcggataaagttgcaggaccacttctgcgctcggcccttccggctggctggtttattgctgataaatctggagccggtgagcgtgggtctcgcggtatcattgcagcactggggccagatggtaagccctcccgtatcgtagttatctacacgacggggagtcaggcaactatggatgaacgaaatagacagatcgctgagataggtgcctcactgattaagcattggtaactgtcagaccaagtttactcatatatactttagattgatttaaaacttcatttttaatttaaaaggatctaggtgaagatcctttttgataatctcatgaccaaaatcccttaacgtgagttttcgttccactgagcgtcagaccccgtagaaaagatcaaaggatcttcttgagatcctttttttctgcgcgtaatctgctgcttgcaaacaaaaaaaccaccgctaccagcggtggtttgtttgccggatcaagagctaccaactctttttccgaaggtaactggcttcagcagagcgcagataccaaatactgttcttctagtgtagccgtagttaggccaccacttcaagaactctgtagcaccgcctacatacctcgctctgctaatcctgttaccagtggctgctgccagtggcgataagtcgtgtcttaccgggttggactcaagacgatagttaccggataaggcgcagcggtcgggctgaacggggggttcgtgcacacagcccagcttggagcgaacgacctacaccgaactgagatacctacagcgtgagctatgagaaagcgccacgcttcccgaagggagaaaggcggacaggtatccggtaagcggcagggtcggaacaggagagcgcacgagggagcttccagggggaaacgcctggtatctttatagtcctgtcgggtttcgccacctctgacttgagcgtcgatttttgtgatgctcgtcaggggggcggagcctatggaaaaacgccagcaacgcggcctttttacggttcctggccttttgctggccttttgctcacatgttctttcctgcgttatcccctgattctgtggataaccgtattaccgcctttgagtgagctgataccgctcgccgcagccgaacgaccgagcgcagcgagtcagtgagcgaggaagcggaagagcgcccaatacgcaaaccgcctctccccgcgcgttggccgattcattaatgcagctggcacgacaggtttcccgactggaaagcgggcagtgagcgcaacgcaattaatgtgagttagctcactcattaggcaccccaggctttacactttatgcttccggctcgtatgttgtgtggaattgtgagcggataacaatttcacacaggaaacagctatgaccatgattacgccaagcgcgcaattaaccctcactaaagggaacaaaagctggagctgcaagcttggccattgcatacgttgtatccatatcataatatgtacatttatattggctcatgtccaacattaccgccatgttgacattgattattgactagttattaatagtaatcaattacggggtcattagttcatagcccatatatggagttccgcgttacataacttacggtaaatggcccgcctggctgaccgcccaacgacccccgcccattgacgtcaataatgacgtatgttcccatagtaacgccaatagggactttccattgacgtcaatgggtggagtatttacggtaaactgcccacttggcagtacatcaagtgtatcatatgccaagtacgccccctattgacgtcaatgacggtaaatggcccgcctggcattatgcccagtacatgaccttatgggactttcctacttggcagtacatctacgtattagtcatcgctattaccatggtgatgcggttttggcagtacatcaatgggcgtggatagcggtttgactcacggggatttccaagtctccaccccattgacgtcaatgggagtttgttttggcaccaaaatcaacgggactttccaaaatgtcgtaacaactccgccccattgacgcaaatgggcggtaggcgtgtacggtgggaggtctatataagcagagctcgtttagtgaaccggggtctctctggttagaccagatctgagcctgggagctctctggctaactagggaacccactgcttaagcctcaataaagcttgccttgagtgcttcaagtagtgtgtgcccgtctgttgtgtgactctggtaactagagatccctcagacccttttagtcagtgtggaaaatctctagcagtggcgcccgaacagggacttgaaagcgaaagggaaaccagaggagctctctcgacgcaggactcggcttgctgaagcgcgcacggcaagaggcgaggggcggcgactggtgagtacgccaaaaattttgactagcggaggctagaaggagagagatgggtgcgagagcgtcagtattaagcgggggagaattagatcgcgatgggaaaaaattcggttaaggccagggggaaagaaaaaatataaattaaaacatatagtatgggcaagcagggagctagaacgattcgcagttaatcctggcctgttagaaacatcagaaggctgtagacaaatactgggacagctacaaccatcccttcagacaggatcagaagaacttagatcattatataatacagtagcaaccctctattgtgtgcatcaaaggatagagataaaagacaccaaggaagctttagacaagatagaggaagagcaaaacaaaagtaagaccaccgcacagcaagcggccgctgatcttcagacctggaggaggagatatgagggacaattggagaagtgaattatataaatataaagtagtaaaaattgaaccattaggagtagcacccaccaaggcaaagagaagagtggtgcagagagaaaaaagagcagtgggaataggagctttgttccttgggttcttgggagcagcaggaagcactatgggcgcagcctcaatgacgctgacggtacaggccagacaattattgtctggtatagtgcagcagcagaacaatttgctgagggctattgaggcgcaacagcatctgttgcaactcacagtctggggcatcaagcagctccaggcaagaatcctggctgtggaaagatacctaaaggatcaacagctcctggggatttggggttgctctggaaaactcatttgcaccactgctgtgccttggaatgctagttggagtaataaatctctggaacagatttggaatcacacgacctggatggagtgggacagagaaattaacaattacacaagcttaatacactccttaattgaagaatcgcaaaaccagcaagaaaagaatgaacaagaattattggaattagataaatgggcaagtttgtggaattggtttaacataacaaattggctgtggtatataaaattattcataatgatagtaggaggcttggtaggtttaagaatagtttttgctgtactttctatagtgaatagagttaggcagggatattcaccattatcgtttcagacccacctcccaaccccgaggggacccgacaggcccgaaggaatagaagaagaaggtggagagagagacagagacagatccattcgattagtgaacggatctcgacggtatcggttaacttttaaaagaaaaggggggattggggggtacagtgcaggggaaagaatagtagacataatagcaacagacatacaaactaaagaattacaaaaacaaattacaaaaattcaaaattttatcgatcacgagactagcctcgagcgtggaggaaaaactgtttcatacagaaggcgtggaggaaaaactgtttcatacagaaggcgtggaggaaaaactgtttcatacagaaggcgtggaggaaaaactgtttcatacagaaggcgtggaggaaaaactgtttcatacagaaggcgtggaggaaaaactgtttcatacagaaggcgtctgcaggagactctagagggtatataatggtttaaacttaagcttggtaccgggcccccgaagacgcgtgccaccatggcctggaccgttctcctcctcggcctcctctctcactgcacaggctctgtgacctcctactttggcaagcttgaatctaaattatcagtcataagaaatttgaatgaccaagttctcttcattgaccaaggaaatcggcctctatttgaagatatgactgattctgactgtagagataatgcaccccggaccatatttattataagtatgtataaagatagccagcctagaggtatggctgtaactatctctgtgaagtgtgagaaaatttcaactctctcctgtgagaacaaaattatttcctttaaggaaatgaatcctcctgataacatcaaggatacaaaaagtgacatcatattctttcagagaagtgtcccaggacatgataataagatgcaatttgaatcttcatcatacgaaggatactttctagcttgtgaaaaagagagagacctttttaaactcattttgaaaaaagaggatgaattgggggatagatctataatgttcactgttcaaaacgaagactagtgtacaagtaatcgaattcccacggggttggggttgcgccttttccaaggcagccctgggtttgcgcagggacgcggctgctctgggcgtggttccgggaaacgcagcggcgccgaccctgggtctcgcacattcttcacgtccgttcgcagcgtcacccggatcttcgccgctacccttgtgggccccccggcgacgcttcctgctccgcccctaagtcgggaaggttccttgcggttcgcggcgtgccggacgtgacaaacggaagccgcacgtctcactagtaccctcgcagacggacagcgccagggagcaatggcagcgcgccgaccgcgatgggctgtggccaatagcggctgctcagcggggcgcgccgagagcagcggccgggaaggggcggtgcgggaggcggggtgtggggcggtagtgtgggccctgttcctgcccgcgcggtgttccgcattctgcaagcctccggagcgcacgtcggcagtcggctccctcgttgaccgaatcaccgacctctctccccagggggatccaccggtcacgtggctagcgccaccnnnnnnnnnnnnnnnnnnnnnnnnnnnnnnnnnnnnnnnnnnnnnnnnnnnnnnnnnnnnnnnnnnnnnnnnnnnnnnnnnnnnnnnnnnnnnnnnnnnnnnnnnnnnnnnnnnnnnnnnnnnnnnnnnnnnnnnnnnnnnnnnnnnnnnnnnnnnnnnnnnnnnnnnnnnnnnnnnnnnnnnnnnnnnnnnnnnnnnnnnnnnnnnnnnnnnnnnnnnnnnnnnnnnnnnnnnnnnnnnnnnnnnnnnnnnnnnnnnnnnnnnnnnnnnnnnnnnnnnnnnnnnnnnnnnnnnnnnnnnnnnnnnnnnnnnnnnnnnnnnnnnnnnnnnnnnnnnnnnnnnnnnnnnnnnnnnnnnnnnnnnnnnnnnnnnnnnnnnnnnnnnnnnnnnnnnnnnnnnnnnnnnnnnnnnnnnnnnnnnnnnnnnnnnnnnnnnnnnnnnnnnnnnnnnnnnnnnnnnnnnnnnnnnnnnnnnnnnnnnnnnnnnnnnnnnnnnnnnnnnnnnnnnnnnnnnnnnnnnnnnnnnnnnnnnnnnnnnnnnnnnnnnnnnnnnnnnnnnnnnnnnnnnnnnnnnnnnnnnnnnnnnnnnnnnnnnnnnnnnnnnnnnnnnnnnnnnnnnnnnnnnnnnnnnnnnnnnnnnnnnnnnnnnnnnnnnnnnnnnnnnnnnnnnnnnnnnnnnnnnnnnnnnnnnnnnnnnnnnnnnnnnnnnnnnnnnnnnnnnnnnnnnnnnnnnnnnnnnnnnnnnnnnnnnnnnnnnnnnnnnnnnnnnnnnnnnnnnnnnnnnnnnnnnnnnnnnnnnnnnnnnnnnnnnnnnnnnnnnnnnnnnnnnnnnnnnnnnnnnnnnnnnnnnnnnnnnnnnnnnnnnnnnnnnnnnnnnnnnnnnnnnnnnnnnnnnnnnnnnnnnnnnnnnnnnnnnnnnnnnnnnnnnnnnnnnnnnnnnnnnnnnnnnnnnnnnnnnnnnnnnnnnnnnnnnnnnnnnnnnnnnnnnnnnnnnnnnnnnnnnnnnnnnnnnnnnnnnnnnnnnnnnnnnnnnnnnnnnnnnnnnnnnnnnnnnnnnnnnnnnnnnnnnnnnnnnnnnnnnnnnnnnnnnnnnnnnnnnnnnnnnnnnnnnnnnnnnnnnnnnnnnnnnnnnnnnnnnnnnnnnnnnnnnnnnnnnnnnnnnnnnnnnnnnnnnnnnnnnnnnnnnnnnnnnnnnnnnnnnnnnnnnnnnnnnnnnnnnnnnnnnnnnnnnnnnnnnnnnnnnnnnnnnnnnnnnnnnnnnnnnnnnnnnnnnnnnnnnnnnnnnnnnnnnnnnnnnnnnnnnnnnnnnnnnnnnnnnnnnnnnnnnnnnnnnnnnnnnnnnnnnnnnnnnnnnnnnnnnnnnnnnnnnnnnnnnnnnnnnnnnnnnnnnnnnnnnnnnnnnnnnnnnnnnnnnnnnnnnnnnnnnnnnnnnnnnnnnnnnnnnnnnnnnnnnnnntaggatccgccggcggccgcgtcgacaatcaacctctggattacaaaatttgtgaaagattgactggtattcttaactatgttgctccttttacgctatgtggatacgctgctttaatgcctttgtatcatgctattgcttcccgtatggctttcattttctcctccttgtataaatcctggttgctgtctctttatgaggagttgtggcccgttgtcaggcaacgtggcgtggtgtgcactgtgtttgctgacgcaacccccactggttggggcattgccaccacctgtcagctcctttccgggactttcgctttccccctccctattgccacggcggaactcatcgccgcctgccttgcccgctgctggacaggggctcggctgttgggcactgacaattccgtggtgttgtcggggaagctgacgtcctttccatggctgctcgcctgtgttgccacctggattctgcgcgggacgtccttctgctacgtcccttcggccctcaatccagcggaccttccttcccgcggcctgctgccggctctgcggcctcttccgcgtcttcgccttcgccctcagacgagtcggatctccctttgggccgcctccccgcctggaattcgagctcggtacctttaagaccaatgacttacaaggcagctgtagatcttagccactttttaaaagaaaaggggggactggaagggctaattcactcccaacgaagacaagatctgctttttgcttgtactgggtctctctggttagaccagatctgagcctgggagctctctggctaactagggaacccactgcttaagcctcaataaagcttgccttgagtgcttcaagtagtgtgtgcccgtctgttgtgtgactctggtaactagagatccctcagacccttttagtcagtgtggaaaatctctagcagtagtagttcatgtcatcttattattcagtatttataacttgcaaagaaatgaatatcagagagtgagaggaacttgtttattgcagcttataatggttacaaataaagcaatagcatcacaaatttcacaaataaagcatttttttcactgcattctagttgtggtttgtccaaactcatcaatgtatcttatcatgtctggctctagctatcccgcccctaactccgcccagttccgcccattctccgccccatggctgactaattttttttatttatgcagaggccgaggccgcctcggcctctgagctattccagaagtagtgaggaggcttttttggaggcctaggcttttgcgtcgagacgtacccaattcgccctatagtgagtcgtattacgcgcgctcactggccgtcgttttacaacgtcgtgactgggaaaaccctggcgttacccaacttaatcgccttgcagcacatccccctttcgccagctggcgtaatagcgaagaggcccgcaccgatcgcccttcccaacagttgcgcagcctgaatggcgaatggcgcgacgcgccctgtagcggcgcattaagcgcggcgggtgtggtggttacgcgcagcgtgaccgctacacttgccagcgccctagcgcccgctcctttcgctttcttcccttcctttctcgccacgttcgccggctttccccgtcaagctctaaatcgggggctccctttagggttccgatttagtgctttacggcacctcgaccccaaaaaacttgattagggtgatggttcacgtagtgggccatcgccctgatagacggtttttcgccctttgacgttggagtccacgttctttaatagtggactcttgttccaaactggaacaacactcaaccctatctcggtctattcttttgatttataagggattttgccgatttcggcctattggttaaaaaatgagctgatttaacaaaaatttaacgcgaattttaacaaaatattaacgtttacaatttcccaggtggcacttttcggggaaatgtgcgcggaacccctatttgtttatttttctaaatacattcaaatatgtatccgctcatgagacaataaccctgataaatgcttcaataatattgaaaaaggaagagtatgagtattcaacatttccgtgtcgcccttattcccttttttgcggcattttgccttcctgtttttgctcacccagaaacgctggtgaaagtaaaagatgctgaagatcagttgggtgcacgagtgggttacatcgaactggatctcaacagcggtaagatccttgagagttttcgccccgaagaacgttttccaatgatgagcacttttaaagttctgctatgtggcgcggtattatcccgtattgacgccgggcaagagcaactcggtcgccgcatacactattctcagaatgacttggttg

SEQ ID NO: 19 - protein, 177 aa, Artificial Sequence; identical to SEQ ID NO: 7
  [CDS]:4430..4963 from SEQ ID NO 18

SEQ ID NO: 20 - DNA, 9684 bp, Artificial Sequence
  pCCL.PPT.NFATmIL2.EGFP.PGK.CAR.wPRE
  misc_signal 2683..2808: /note="HIV-1 packaging signal"
  misc_feature 3302..3543: /note="RRE: rev response element of HIV-1"
  misc_feature 4030..4147: /note="cPPT/CTScPPT/CTS: central polypurine tract and central termination sequence of HIV-1"
  promoter 4178..4414: /note="6x NFAT"
  promoter 4421..4540: /note="mIL2 promoter including TATA box"
  CDS 4559..5278: /note="eGFP" /transl_table=1
  promoter 5287..5802: /note="PGK promoter"
  gene 5834..7288: /gene="placeholder for CAR"
  misc_signal 7315..7903: /note="wPRE: woodchuck hepatitis virus posttranscriptional regulatory element"
agtactcaccagtcacagaaaagcatcttacggatggcatgacagtaagagaattatgcagtgctgccataaccatgagtgataacactgcggccaacttacttctgacaacgatcggaggaccgaaggagctaaccgcttttttgcacaacatgggggatcatgtaactcgccttgatcgttgggaaccggagctgaatgaagccataccaaacgacgagcgtgacaccacgatgcctgtagcaatggcaacaacgttgcgcaaactattaactggcgaactacttactctagcttcccggcaacaattaatagactggatggaggcggataaagttgcaggaccacttctgcgctcggcccttccggctggctggtttattgctgataaatctggagccggtgagcgtgggtctcgcggtatcattgcagcactggggccagatggtaagccctcccgtatcgtagttatctacacgacggggagtcaggcaactatggatgaacgaaatagacagatcgctgagataggtgcctcactgattaagcattggtaactgtcagaccaagtttactcatatatactttagattgatttaaaacttcatttttaatttaaaaggatctaggtgaagatcctttttgataatctcatgaccaaaatcccttaacgtgagttttcgttccactgagcgtcagaccccgtagaaaagatcaaaggatcttcttgagatcctttttttctgcgcgtaatctgctgcttgcaaacaaaaaaaccaccgctaccagcggtggtttgtttgccggatcaagagctaccaactctttttccgaaggtaactggcttcagcagagcgcagataccaaatactgttcttctagtgtagccgtagttaggccaccacttcaagaactctgtagcaccgcctacatacctcgctctgctaatcctgttaccagtggctgctgccagtggcgataagtcgtgtcttaccgggttggactcaagacgatagttaccggataaggcgcagcggtcgggctgaacggggggttcgtgcacacagcccagcttggagcgaacgacctacaccgaactgagatacctacagcgtgagctatgagaaagcgccacgcttcccgaagggagaaaggcggacaggtatccggtaagcggcagggtcggaacaggagagcgcacgagggagcttccagggggaaacgcctggtatctttatagtcctgtcgggtttcgccacctctgacttgagcgtcgatttttgtgatgctcgtcaggggggcggagcctatggaaaaacgccagcaacgcggcctttttacggttcctggccttttgctggccttttgctcacatgttctttcctgcgttatcccctgattctgtggataaccgtattaccgcctttgagtgagctgataccgctcgccgcagccgaacgaccgagcgcagcgagtcagtgagcgaggaagcggaagagcgcccaatacgcaaaccgcctctccccgcgcgttggccgattcattaatgcagctggcacgacaggtttcccgactggaaagcgggcagtgagcgcaacgcaattaatgtgagttagctcactcattaggcaccccaggctttacactttatgcttccggctcgtatgttgtgtggaattgtgagcggataacaatttcacacaggaaacagctatgaccatgattacgccaagcgcgcaattaaccctcactaaagggaacaaaagctggagctgcaagcttggccattgcatacgttgtatccatatcataatatgtacatttatattggctcatgtccaacattaccgccatgttgacattgattattgactagttattaatagtaatcaattacggggtcattagttcatagcccatatatggagttccgcgttacataacttacggtaaatggcccgcctggctgaccgcccaacgacccccgcccattgacgtcaataatgacgtatgttcccatagtaacgccaatagggactttccattgacgtcaatgggtggagtatttacggtaaactgcccacttggcagtacatcaagtgtatcatatgccaagtacgccccctattgacgtcaatgacggtaaatggcccgcctggcattatgcccagtacatgaccttatgggactttcctacttggcagtacatctacgtattagtcatcgctattaccatggtgatgcggttttggcagtacatcaatgggcgtggatagcggtttgactcacggggatttccaagtctccaccccattgacgtcaatgggagtttgttttggcaccaaaatcaacgggactttccaaaatgtcgtaacaactccgccccattgacgcaaatgggcggtaggcgtgtacggtgggaggtctatataagcagagctcgtttagtgaaccggggtctctctggttagaccagatctgagcctgggagctctctggctaactagggaacccactgcttaagcctcaataaagcttgccttgagtgcttcaagtagtgtgtgcccgtctgttgtgtgactctggtaactagagatccctcagacccttttagtcagtgtggaaaatctctagcagtggcgcccgaacagggacttgaaagcgaaagggaaaccagaggagctctctcgacgcaggactcggcttgctgaagcgcgcacggcaagaggcgaggggcggcgactggtgagtacgccaaaaattttgactagcggaggctagaaggagagagatgggtgcgagagcgtcagtattaagcgggggagaattagatcgcgatgggaaaaaattcggttaaggccagggggaaagaaaaaatataaattaaaacatatagtatgggcaagcagggagctagaacgattcgcagttaatcctggcctgttagaaacatcagaaggctgtagacaaatactgggacagctacaaccatcccttcagacaggatcagaagaacttagatcattatataatacagtagcaaccctctattgtgtgcatcaaaggatagagataaaagacaccaaggaagctttagacaagatagaggaagagcaaaacaaaagtaagaccaccgcacagcaagcggccgctgatcttcagacctggaggaggagatatgagggacaattggagaagtgaattatataaatataaagtagtaaaaattgaaccattaggagtagcacccaccaaggcaaagagaagagtggtgcagagagaaaaaagagcagtgggaataggagctttgttccttgggttcttgggagcagcaggaagcactatgggcgcagcctcaatgacgctgacggtacaggccagacaattattgtctggtatagtgcagcagcagaacaatttgctgagggctattgaggcgcaacagcatctgttgcaactcacagtctggggcatcaagcagctccaggcaagaatcctggctgtggaaagatacctaaaggatcaacagctcctggggatttggggttgctctggaaaactcatttgcaccactgctgtgccttggaatgctagttggagtaataaatctctggaacagatttggaatcacacgacctggatggagtgggacagagaaattaacaattacacaagcttaatacactccttaattgaagaatcgcaaaaccagcaagaaaagaatgaacaagaattattggaattagataaatgggcaagtttgtggaattggtttaacataacaaattggctgtggtatataaaattattcataatgatagtaggaggcttggtaggtttaagaatagtttttgctgtactttctatagtgaatagagttaggcagggatattcaccattatcgtttcagacccacctcccaaccccgaggggacccgacaggcccgaaggaatagaagaagaaggtggagagagagacagagacagatccattcgattagtgaacggatctcgacggtatcggttaacttttaaaagaaaaggggggattggggggtacagtgcaggggaaagaatagtagacataatagcaacagacatacaaactaaagaattacaaaaacaaattacaaaaattcaaaattttatcgatcacgagactagcctcgacagcgctgatatcgaattaggaggaaaaactgtttcatacagaaggcgtcaattaggaggaaaaactgtttcatacagaaggcgtcaattaggaggaaaaactgtttcatacagaaggcgtcaattggtcccatcgaattaggaggaaaaactgtttcatacagaaggcgtcaattaggaggaaaaactgtttcatacagaaggcgtcaattaggaggaaaaactgtttcatacagaaggcgtcaattggtcccgggacattttgacacccccataatatttttccagaattaacagtataaattgcatctcttgttcaagagttccctatcactctctttaatcactactcacagtaacctcaactcctggatccacgcgtgccaccatggtgagcaagggcgaggagctgttcaccggggtggtgcccatcctggtcgagctggacggcgacgtaaacggccacaagttcagcgtgtccggcgagggcgagggcgatgccacctacggcaagctgaccctgaagttcatctgcaccaccggcaagctgcccgtgccctggcccaccctcgtgaccaccctgacctacggcgtgcagtgcttcagccgctaccccgaccacatgaagcagcacgacttcttcaagtccgccatgcccgaaggctacgtccaggagcgcaccatcttcttcaaggacgacggcaactacaagacccgcgccgaggtgaagttcgagggcgacaccctggtgaaccgcatcgagctgaagggcatcgacttcaaggaggacggcaacatcctggggcacaagctggagtacaactacaacagccacaacgtctatatcatggccgacaagcagaagaacggcatcaaggtgaacttcaagatccgccacaacatcgaggacggcagcgtgcagctcgccgaccactaccagcagaacacccccatcggcgacggccccgtgctgctgcccgacaaccactacctgagcacccagtccgccctgagcaaagaccccaacgagaagcgcgatcacatggtcctgctggagttcgtgaccgccgccgggatcactctcggcatggacgagctgtacaagtaatcgaattcccacggggttggggttgcgccttttccaaggcagccctgggtttgcgcagggacgcggctgctctgggcgtggttccgggaaacgcagcggcgccgaccctgggtctcgcacattcttcacgtccgttcgcagcgtcacccggatcttcgccgctacccttgtgggccccccggcgacgcttcctgctccgcccctaagtcgggaaggttccttgcggttcgcggcgtgccggacgtgacaaacggaagccgcacgtctcactagtaccctcgcagacggacagcgccagggagcaatggcagcgcgccgaccgcgatgggctgtggccaatagcggctgctcagcggggcgcgccgagagcagcggccgggaaggggcggtgcgggaggcggggtgtggggcggtagtgtgggccctgttcctgcccgcgcggtgttccgcattctgcaagcctccggagcgcacgtcggcagtcggctccctcgttgaccgaatcaccgacctctctccccagggggatccaccggtcacgtggctagcgccaccnnnnnnnnnnnnnnnnnnnnnnnnnnnnnnnnnnnnnnnnnnnnnnnnnnnnnnnnnnnnnnnnnnnnnnnnnnnnnnnnnnnnnnnnnnnnnnnnnnnnnnnnnnnnnnnnnnnnnnnnnnnnnnnnnnnnnnnnnnnnnnnnnnnnnnnnnnnnnnnnnnnnnnnnnnnnnnnnnnnnnnnnnnnnnnnnnnnnnnnnnnnnnnnnnnnnnnnnnnnnnnnnnnnnnnnnnnnnnnnnnnnnnnnnnnnnnnnnnnnnnnnnnnnnnnnnnnnnnnnnnnnnnnnnnnnnnnnnnnnnnnnnnnnnnnnnnnnnnnnnnnnnnnnnnnnnnnnnnnnnnnnnnnnnnnnnnnnnnnnnnnnnnnnnnnnnnnnnnnnnnnnnnnnnnnnnnnnnnnnnnnnnnnnnnnnnnnnnnnnnnnnnnnnnnnnnnnnnnnnnnnnnnnnnnnnnnnnnnnnnnnnnnnnnnnnnnnnnnnnnnnnnnnnnnnnnnnnnnnnnnnnnnnnnnnnnnnnnnnnnnnnnnnnnnnnnnnnnnnnnnnnnnnnnnnnnnnnnnnnnnnnnnnnnnnnnnnnnnnnnnnnnnnnnnnnnnnnnnnnnnnnnnnnnnnnnnnnnnnnnnnnnnnnnnnnnnnnnnnnnnnnnnnnnnnnnnnnnnnnnnnnnnnnnnnnnnnnnnnnnnnnnnnnnnnnnnnnnnnnnnnnnnnnnnnnnnnnnnnnnnnnnnnnnnnnnnnnnnnnnnnnnnnnnnnnnnnnnnnnnnnnnnnnnnnnnnnnnnnnnnnnnnnnnnnnnnnnnnnnnnnnnnnnnnnnnnnnnnnnnnnnnnnnnnnnnnnnnnnnnnnnnnnnnnnnnnnnnnnnnnnnnnnnnnnnnnnnnnnnnnnnnnnnnnnnnnnnnnnnnnnnnnnnnnnnnnnnnnnnnnnnnnnnnnnnnnnnnnnnnnnnnnnnnnnnnnnnnnnnnnnnnnnnnnnnnnnnnnnnnnnnnnnnnnnnnnnnnnnnnnnnnnnnnnnnnnnnnnnnnnnnnnnnnnnnnnnnnnnnnnnnnnnnnnnnnnnnnnnnnnnnnnnnnnnnnnnnnnnnnnnnnnnnnnnnnnnnnnnnnnnnnnnnnnnnnnnnnnnnnnnnnnnnnnnnnnnnnnnnnnnnnnnnnnnnnnnnnnnnnnnnnnnnnnnnnnnnnnnnnnnnnnnnnnnnnnnnnnnnnnnnnnnnnnnnnnnnnnnnnnnnnnnnnnnnnnnnnnnnnnnnnnnnnnnnnnnnnnnnnnnnnnnnnnnnnnnnnnnnnnnnnnnnnnnnnnnnnnnnnnnnnnnnnnnnnnnnnnnnnnnnnnnnnnnnnnnnnnnnnnnnnnnnnnnnnnnnnnnnnnnnnnnnnnnnnnnnnnnnnnnnnnnnnnnnnnnnnnnnnnnnnnnnnnnnnnnnnnnnnnnnnnnnnnnnnnnnnnnnnnnnnnnnnnnnnnnntaggatccgccggcggccgcgtcgacaatcaacctctggattacaaaatttgtgaaagattgactggtattcttaactatgttgctccttttacgctatgtggatacgctgctttaatgcctttgtatcatgctattgcttcccgtatggctttcattttctcctccttgtataaatcctggttgctgtctctttatgaggagttgtggcccgttgtcaggcaacgtggcgtggtgtgcactgtgtttgctgacgcaacccccactggttggggcattgccaccacctgtcagctcctttccgggactttcgctttccccctccctattgccacggcggaactcatcgccgcctgccttgcccgctgctggacaggggctcggctgttgggcactgacaattccgtggtgttgtcggggaagctgacgtcctttccatggctgctcgcctgtgttgccacctggattctgcgcgggacgtccttctgctacgtcccttcggccctcaatccagcggaccttccttcccgcggcctgctgccggctctgcggcctcttccgcgtcttcgccttcgccctcagacgagtcggatctccctttgggccgcctccccgcctggaattcgagctcggtacctttaagaccaatgacttacaaggcagctgtagatcttagccactttttaaaagaaaaggggggactggaagggctaattcactcccaacgaagacaagatctgctttttgcttgtactgggtctctctggttagaccagatctgagcctgggagctctctggctaactagggaacccactgcttaagcctcaataaagcttgccttgagtgcttcaagtagtgtgtgcccgtctgttgtgtgactctggtaactagagatccctcagacccttttagtcagtgtggaaaatctctagcagtagtagttcatgtcatcttattattcagtatttataacttgcaaagaaatgaatatcagagagtgagaggaacttgtttattgcagcttataatggttacaaataaagcaatagcatcacaaatttcacaaataaagcatttttttcactgcattctagttgtggtttgtccaaactcatcaatgtatcttatcatgtctggctctagctatcccgcccctaactccgcccagttccgcccattctccgccccatggctgactaattttttttatttatgcagaggccgaggccgcctcggcctctgagctattccagaagtagtgaggaggcttttttggaggcctaggcttttgcgtcgagacgtacccaattcgccctatagtgagtcgtattacgcgcgctcactggccgtcgttttacaacgtcgtgactgggaaaaccctggcgttacccaacttaatcgccttgcagcacatccccctttcgccagctggcgtaatagcgaagaggcccgcaccgatcgcccttcccaacagttgcgcagcctgaatggcgaatggcgcgacgcgccctgtagcggcgcattaagcgcggcgggtgtggtggttacgcgcagcgtgaccgctacacttgccagcgccctagcgcccgctcctttcgctttcttcccttcctttctcgccacgttcgccggctttccccgtcaagctctaaatcgggggctccctttagggttccgatttagtgctttacggcacctcgaccccaaaaaacttgattagggtgatggttcacgtagtgggccatcgccctgatagacggtttttcgccctttgacgttggagtccacgttctttaatagtggactcttgttccaaactggaacaacactcaaccctatctcggtctattcttttgatttataagggattttgccgatttcggcctattggttaaaaaatgagctgatttaacaaaaatttaacgcgaattttaacaaaatattaacgtttacaatttcccaggtggcacttttcggggaaatgtgcgcggaacccctatttgtttatttttctaaatacattcaaatatgtatccgctcatgagacaataaccctgataaatgcttcaataatattgaaaaaggaagagtatgagtattcaacatttccgtgtcgcccttattcccttttttgcggcattttgccttcctgtttttgctcacccagaaacgctggtgaaagtaaaagatgctgaagatcagttgggtgcacgagtgggttacatcgaactggatctcaacagcggtaagatccttgagagttttcgccccgaagaacgttttccaatgatgagcacttttaaagttctgctatgtggcgcggtattatcccgtattgacgccgggcaagagcaactcggtcgccgcatacactattctcagaatgacttggttg

SEQ ID NO: 21 - protein, 239 aa, Artificial Sequence; identical to SEQ ID NO: 9
  [CDS]:4559..5278 from SEQ ID NO 20

SEQ ID NO: 22 - DNA, 10598 bp, Artificial Sequence
  pCCL.PPT.NFATmIL2.humanIL12.PGK.CAR.wPRE
  misc_signal 2683..2808: /note="HIV-1 psi: packaging signal of human immunodeficiency virus type 1"
  misc_signal 3302..3543: /note="RRE: rev response element of HIV-1"
  misc_feature 4030..4147: /note="cPPT/CTScPPT/CTS: central polypurine tract and central termination sequence of HIV-1"
  promoter 4178..4414: /note="6 x NFAT"
  promoter 4421..4540: /note="mIL2 promoter"
  CDS 4559..6181: /gene="sc Il12 humanized codon usage" /transl_table=1
  promoter 6201..6716: /note="PGK promoter"
  gene 6748..8202: /gene="placeholder for CAR"
  misc_signal 8229..8817: /note="wPRE: woodchuck hepatitis virus posttranscriptional regulatory element"
agtactcaccagtcacagaaaagcatcttacggatggcatgacagtaagagaattatgcagtgctgccataaccatgagtgataacactgcggccaacttacttctgacaacgatcggaggaccgaaggagctaaccgcttttttgcacaacatgggggatcatgtaactcgccttgatcgttgggaaccggagctgaatgaagccataccaaacgacgagcgtgacaccacgatgcctgtagcaatggcaacaacgttgcgcaaactattaactggcgaactacttactctagcttcccggcaacaattaatagactggatggaggcggataaagttgcaggaccacttctgcgctcggcccttccggctggctggtttattgctgataaatctggagccggtgagcgtgggtctcgcggtatcattgcagcactggggccagatggtaagccctcccgtatcgtagttatctacacgacggggagtcaggcaactatggatgaacgaaatagacagatcgctgagataggtgcctcactgattaagcattggtaactgtcagaccaagtttactcatatatactttagattgatttaaaacttcatttttaatttaaaaggatctaggtgaagatcctttttgataatctcatgaccaaaatcccttaacgtgagttttcgttccactgagcgtcagaccccgtagaaaagatcaaaggatcttcttgagatcctttttttctgcgcgtaatctgctgcttgcaaacaaaaaaaccaccgctaccagcggtggtttgtttgccggatcaagagctaccaactctttttccgaaggtaactggcttcagcagagcgcagataccaaatactgttcttctagtgtagccgtagttaggccaccacttcaagaactctgtagcaccgcctacatacctcgctctgctaatcctgttaccagtggctgctgccagtggcgataagtcgtgtcttaccgggttggactcaagacgatagttaccggataaggcgcagcggtcgggctgaacggggggttcgtgcacacagcccagcttggagcgaacgacctacaccgaactgagatacctacagcgtgagctatgagaaagcgccacgcttcccgaagggagaaaggcggacaggtatccggtaagcggcagggtcggaacaggagagcgcacgagggagcttccagggggaaacgcctggtatctttatagtcctgtcgggtttcgccacctctgacttgagcgtcgatttttgtgatgctcgtcaggggggcggagcctatggaaaaacgccagcaacgcggcctttttacggttcctggccttttgctggccttttgctcacatgttctttcctgcgttatcccctgattctgtggataaccgtattaccgcctttgagtgagctgataccgctcgccgcagccgaacgaccgagcgcagcgagtcagtgagcgaggaagcggaagagcgcccaatacgcaaaccgcctctccccgcgcgttggccgattcattaatgcagctggcacgacaggtttcccgactggaaagcgggcagtgagcgcaacgcaattaatgtgagttagctcactcattaggcaccccaggctttacactttatgcttccggctcgtatgttgtgtggaattgtgagcggataacaatttcacacaggaaacagctatgaccatgattacgccaagcgcgcaattaaccctcactaaagggaacaaaagctggagctgcaagcttggccattgcatacgttgtatccatatcataatatgtacatttatattggctcatgtccaacattaccgccatgttgacattgattattgactagttattaatagtaatcaattacggggtcattagttcatagcccatatatggagttccgcgttacataacttacggtaaatggcccgcctggctgaccgcccaacgacccccgcccattgacgtcaataatgacgtatgttcccatagtaacgccaatagggactttccattgacgtcaatgggtggagtatttacggtaaactgcccacttggcagtacatcaagtgtatcatatgccaagtacgccccctattgacgtcaatgacggtaaatggcccgcctggcattatgcccagtacatgaccttatgggactttcctacttggcagtacatctacgtattagtcatcgctattaccatggtgatgcggttttggcagtacatcaatgggcgtggatagcggtttgactcacggggatttccaagtctccaccccattgacgtcaatgggagtttgttttggcaccaaaatcaacgggactttccaaaatgtcgtaacaactccgccccattgacgcaaatgggcggtaggcgtgtacggtgggaggtctatataagcagagctcgtttagtgaaccggggtctctctggttagaccagatctgagcctgggagctctctggctaactagggaacccactgcttaagcctcaataaagcttgccttgagtgcttcaagtagtgtgtgcccgtctgttgtgtgactctggtaactagagatccctcagacccttttagtcagtgtggaaaatctctagcagtggcgcccgaacagggacttgaaagcgaaagggaaaccagaggagctctctcgacgcaggactcggcttgctgaagcgcgcacggcaagaggcgaggggcggcgactggtgagtacgccaaaaattttgactagcggaggctagaaggagagagatgggtgcgagagcgtcagtattaagcgggggagaattagatcgcgatgggaaaaaattcggttaaggccagggggaaagaaaaaatataaattaaaacatatagtatgggcaagcagggagctagaacgattcgcagttaatcctggcctgttagaaacatcagaaggctgtagacaaatactgggacagctacaaccatcccttcagacaggatcagaagaacttagatcattatataatacagtagcaaccctctattgtgtgcatcaaaggatagagataaaagacaccaaggaagctttagacaagatagaggaagagcaaaacaaaagtaagaccaccgcacagcaagcggccgctgatcttcagacctggaggaggagatatgagggacaattggagaagtgaattatataaatataaagtagtaaaaattgaaccattaggagtagcacccaccaaggcaaagagaagagtggtgcagagagaaaaaagagcagtgggaataggagctttgttccttgggttcttgggagcagcaggaagcactatgggcgcagcctcaatgacgctgacggtacaggccagacaattattgtctggtatagtgcagcagcagaacaatttgctgagggctattgaggcgcaacagcatctgttgcaactcacagtctggggcatcaagcagctccaggcaagaatcctggctgtggaaagatacctaaaggatcaacagctcctggggatttggggttgctctggaaaactcatttgcaccactgctgtgccttggaatgctagttggagtaataaatctctggaacagatttggaatcacacgacctggatggagtgggacagagaaattaacaattacacaagcttaatacactccttaattgaagaatcgcaaaaccagcaagaaaagaatgaacaagaattattggaattagataaatgggcaagtttgtggaattggtttaacataacaaattggctgtggtatataaaattattcataatgatagtaggaggcttggtaggtttaagaatagtttttgctgtactttctatagtgaatagagttaggcagggatattcaccattatcgtttcagacccacctcccaaccccgaggggacccgacaggcccgaaggaatagaagaagaaggtggagagagagacagagacagatccattcgattagtgaacggatctcgacggtatcggttaacttttaaaagaaaaggggggattggggggtacagtgcaggggaaagaatagtagacataatagcaacagacatacaaactaaagaattacaaaaacaaattacaaaaattcaaaattttatcgatcacgagactagcctcgacagcgctgatatcgaattaggaggaaaaactgtttcatacagaaggcgtcaattaggaggaaaaactgtttcatacagaaggcgtcaattaggaggaaaaactgtttcatacagaaggcgtcaattggtcccatcgaattaggaggaaaaactgtttcatacagaaggcgtcaattaggaggaaaaactgtttcatacagaaggcgtcaattaggaggaaaaactgtttcatacagaaggcgtcaattggtcccgggacattttgacacccccataatatttttccagaattaacagtataaattgcatctcttgttcaagagttccctatcactctctttaatcactactcacagtaacctcaactcctggatccacgcgtgccaccatgtgtcaccagcagctggtcatcagctggttcagcctggtgttcctggcctctcctctggtggccatctgggagctgaagaaagacgtgtacgtggtggaactggactggtatcccgatgctcctggcgagatggtggtgctgacctgcgatacccctgaagaggacggcatcacctggacactggatcagtctagcgaggtgctcggcagcggcaagaccctgaccatccaagtgaaagagtttggcgacgccggccagtacacctgtcacaaaggcggagaagtgctgagccacagcctgctgctgctccacaagaaagaggatggcatttggagcaccgacatcctgaaggaccagaaagagcccaagaacaagaccttcctgagatgcgaggccaagaactacagcggccggttcacatgttggtggctgaccaccatcagcaccgacctgaccttcagcgtgaagtccagcagaggcagcagtgatcctcagggcgttacatgtggcgccgctacactgtctgccgaaagagtgcggggcgacaacaaagaatacgagtacagcgtggaatgccaagaggacagcgcctgtccagccgccgaagagtctctgcctatcgaagtgatggtggacgccgtgcacaagctgaagtacgagaactacacctccagctttttcatccgggacatcatcaagcccgatcctccaaagaacctgcagctgaagcctctgaagaacagcagacaggtggaagtgtcctgggagtaccccgacacctggtctacaccccacagctacttcagcctgaccttttgcgtgcaagtgcagggcaagtccaagcgcgagaaaaaggaccgggtgttcaccgacaagaccagcgccaccgtgatctgcagaaagaacgccagcatcagcgtcagagcccaggaccgctactacagcagctcttggagcgaatgggccagcgtgccatgttctggtggcggaggatctggcggaggtggaagcggcggaggcggatctagaaatctgcctgtggccactcctgatcctggcatgttcccttgtctgcaccacagccagaacctgctgagagccgtgtccaacatgctgcagaaggccagacagaccctggaattctacccctgcaccagcgaggaaatcgaccacgaggacatcaccaaggataagaccagtaccgtggaagcctgcctgcctctggaactgaccaagaacgagagctgcctgaacagccgggaaaccagcttcatcaccaacggctcttgcctggccagcagaaagacctccttcatgatggccctgtgcctgagcagcatctacgaggacctgaagatgtaccaggtggaattcaagaccatgaacgccaagctgctgatggaccccaagcggcagatcttcctggaccagaatatgctggccgtgatcgacgagctgatgcaggccctgaacttcaacagcgagacagtgccccagaagtctagcctggaagaacccgacttctacaagaccaagatcaagctgtgcatcctgctgcacgccttccgcatcagagccgtgaccatcgatagagtgatgagctacctgaacgcctcctgatgtacaagtaatcgaattcccacggggttggggttgcgccttttccaaggcagccctgggtttgcgcagggacgcggctgctctgggcgtggttccgggaaacgcagcggcgccgaccctgggtctcgcacattcttcacgtccgttcgcagcgtcacccggatcttcgccgctacccttgtgggccccccggcgacgcttcctgctccgcccctaagtcgggaaggttccttgcggttcgcggcgtgccggacgtgacaaacggaagccgcacgtctcactagtaccctcgcagacggacagcgccagggagcaatggcagcgcgccgaccgcgatgggctgtggccaatagcggctgctcagcggggcgcgccgagagcagcggccgggaaggggcggtgcgggaggcggggtgtggggcggtagtgtgggccctgttcctgcccgcgcggtgttccgcattctgcaagcctccggagcgcacgtcggcagtcggctccctcgttgaccgaatcaccgacctctctccccagggggatccaccggtcacgtggctagcgccaccnnnnnnnnnnnnnnnnnnnnnnnnnnnnnnnnnnnnnnnnnnnnnnnnnnnnnnnnnnnnnnnnnnnnnnnnnnnnnnnnnnnnnnnnnnnnnnnnnnnnnnnnnnnnnnnnnnnnnnnnnnnnnnnnnnnnnnnnnnnnnnnnnnnnnnnnnnnnnnnnnnnnnnnnnnnnnnnnnnnnnnnnnnnnnnnnnnnnnnnnnnnnnnnnnnnnnnnnnnnnnnnnnnnnnnnnnnnnnnnnnnnnnnnnnnnnnnnnnnnnnnnnnnnnnnnnnnnnnnnnnnnnnnnnnnnnnnnnnnnnnnnnnnnnnnnnnnnnnnnnnnnnnnnnnnnnnnnnnnnnnnnnnnnnnnnnnnnnnnnnnnnnnnnnnnnnnnnnnnnnnnnnnnnnnnnnnnnnnnnnnnnnnnnnnnnnnnnnnnnnnnnnnnnnnnnnnnnnnnnnnnnnnnnnnnnnnnnnnnnnnnnnnnnnnnnnnnnnnnnnnnnnnnnnnnnnnnnnnnnnnnnnnnnnnnnnnnnnnnnnnnnnnnnnnnnnnnnnnnnnnnnnnnnnnnnnnnnnnnnnnnnnnnnnnnnnnnnnnnnnnnnnnnnnnnnnnnnnnnnnnnnnnnnnnnnnnnnnnnnnnnnnnnnnnnnnnnnnnnnnnnnnnnnnnnnnnnnnnnnnnnnnnnnnnnnnnnnnnnnnnnnnnnnnnnnnnnnnnnnnnnnnnnnnnnnnnnnnnnnnnnnnnnnnnnnnnnnnnnnnnnnnnnnnnnnnnnnnnnnnnnnnnnnnnnnnnnnnnnnnnnnnnnnnnnnnnnnnnnnnnnnnnnnnnnnnnnnnnnnnnnnnnnnnnnnnnnnnnnnnnnnnnnnnnnnnnnnnnnnnnnnnnnnnnnnnnnnnnnnnnnnnnnnnnnnnnnnnnnnnnnnnnnnnnnnnnnnnnnnnnnnnnnnnnnnnnnnnnnnnnnnnnnnnnnnnnnnnnnnnnnnnnnnnnnnnnnnnnnnnnnnnnnnnnnnnnnnnnnnnnnnnnnnnnnnnnnnnnnnnnnnnnnnnnnnnnnnnnnnnnnnnnnnnnnnnnnnnnnnnnnnnnnnnnnnnnnnnnnnnnnnnnnnnnnnnnnnnnnnnnnnnnnnnnnnnnnnnnnnnnnnnnnnnnnnnnnnnnnnnnnnnnnnnnnnnnnnnnnnnnnnnnnnnnnnnnnnnnnnnnnnnnnnnnnnnnnnnnnnnnnnnnnnnnnnnnnnnnnnnnnnnnnnnnnnnnnnnnnnnnnnnnnnnnnnnnnnnnnnnnnnnnnnnnnnnnnnnnnnnnnnnnnnnnnnnnnnnnnnnnnnnnnnnnnnnnnnnnnnnnnnnnnnnnnnnnnnnnnnnnnnnnnnnnnnnnnnnnnnnnnnnnnnnnnnnnnnnnnnnnnnnnnnnnnnnnnnnnnnnnnnnnnnnnnnnnnnnnnnnnnnnnnnnnnnnnnnnnnnnnnnnnnnnnnnnnnntaggatccgccggcggccgcgtcgacaatcaacctctggattacaaaatttgtgaaagattgactggtattcttaactatgttgctccttttacgctatgtggatacgctgctttaatgcctttgtatcatgctattgcttcccgtatggctttcattttctcctccttgtataaatcctggttgctgtctctttatgaggagttgtggcccgttgtcaggcaacgtggcgtggtgtgcactgtgtttgctgacgcaacccccactggttggggcattgccaccacctgtcagctcctttccgggactttcgctttccccctccctattgccacggcggaactcatcgccgcctgccttgcccgctgctggacaggggctcggctgttgggcactgacaattccgtggtgttgtcggggaagctgacgtcctttccatggctgctcgcctgtgttgccacctggattctgcgcgggacgtccttctgctacgtcccttcggccctcaatccagcggaccttccttcccgcggcctgctgccggctctgcggcctcttccgcgtcttcgccttcgccctcagacgagtcggatctccctttgggccgcctccccgcctggaattcgagctcggtacctttaagaccaatgacttacaaggcagctgtagatcttagccactttttaaaagaaaaggggggactggaagggctaattcactcccaacgaagacaagatctgctttttgcttgtactgggtctctctggttagaccagatctgagcctgggagctctctggctaactagggaacccactgcttaagcctcaataaagcttgccttgagtgcttcaagtagtgtgtgcccgtctgttgtgtgactctggtaactagagatccctcagacccttttagtcagtgtggaaaatctctagcagtagtagttcatgtcatcttattattcagtatttataacttgcaaagaaatgaatatcagagagtgagaggaacttgtttattgcagcttataatggttacaaataaagcaatagcatcacaaatttcacaaataaagcatttttttcactgcattctagttgtggtttgtccaaactcatcaatgtatcttatcatgtctggctctagctatcccgcccctaactccgcccagttccgcccattctccgccccatggctgactaattttttttatttatgcagaggccgaggccgcctcggcctctgagctattccagaagtagtgaggaggcttttttggaggcctaggcttttgcgtcgagacgtacccaattcgccctatagtgagtcgtattacgcgcgctcactggccgtcgttttacaacgtcgtgactgggaaaaccctggcgttacccaacttaatcgccttgcagcacatccccctttcgccagctggcgtaatagcgaagaggcccgcaccgatcgcccttcccaacagttgcgcagcctgaatggcgaatggcgcgacgcgccctgtagcggcgcattaagcgcggcgggtgtggtggttacgcgcagcgtgaccgctacacttgccagcgccctagcgcccgctcctttcgctttcttcccttcctttctcgccacgttcgccggctttccccgtcaagctctaaatcgggggctccctttagggttccgatttagtgctttacggcacctcgaccccaaaaaacttgattagggtgatggttcacgtagtgggccatcgccctgatagacggtttttcgccctttgacgttggagtccacgttctttaatagtggactcttgttccaaactggaacaacactcaaccctatctcggtctattcttttgatttataagggattttgccgatttcggcctattggttaaaaaatgagctgatttaacaaaaatttaacgcgaattttaacaaaatattaacgtttacaatttcccaggtggcacttttcggggaaatgtgcgcggaacccctatttgtttatttttctaaatacattcaaatatgtatccgctcatgagacaataaccctgataaatgcttcaataatattgaaaaaggaagagtatgagtattcaacatttccgtgtcgcccttattcccttttttgcggcattttgccttcctgtttttgctcacccagaaacgctggtgaaagtaaaagatgctgaagatcagttgggtgcacgagtgggttacatcgaactggatctcaacagcggtaagatccttgagagttttcgccccgaagaacgttttccaatgatgagcacttttaaagttctgctatgtggcgcggtattatcccgtattgacgccgggcaagagcaactcggtcgccgcatacactattctcagaatgacttggttg

SEQ ID NO: 23 - protein, 540 aa, Artificial Sequence; identical to SEQ ID NO: 5
  [CDS]:4559..6181 from SEQ ID NO 22

SEQ ID NO: 24 - DNA, 9476 bp, Artificial Sequence
  pCCL.PPT.NFκBenhsyn.EGFP.PGK.CAR.wPRE
  misc_signal 2683..2808: /note="HIV-1 psi packaging signal of human immunodeficiency virus type 1"
  misc_feature 3301..3534: /note="RRE: Rev response element (RRE) of HIV-1 allows for Rev-dependent mRNA export from the nucleus to the cytoplasm"
  misc_feature 4030..4147: /note="cPPT/CTS: central polypurine tract and central termination sequence of HIV-1"
  promoter 4172..4275: /function="NFκBenhsyn"
  misc_feature 4284..4338: /note="promoter section enhsyn"
  CDS 4351..5070: /gene="eGFP" /transl_table=1
  gene 5626..7080: /gene="CAR"
  misc_feature 7107..7695: /note="WPRE: woodchuck hepatitis virus posttranscriptional regulatory element"
agtactcaccagtcacagaaaagcatcttacggatggcatgacagtaagagaattatgcagtgctgccataaccatgagtgataacactgcggccaacttacttctgacaacgatcggaggaccgaaggagctaaccgcttttttgcacaacatgggggatcatgtaactcgccttgatcgttgggaaccggagctgaatgaagccataccaaacgacgagcgtgacaccacgatgcctgtagcaatggcaacaacgttgcgcaaactattaactggcgaactacttactctagcttcccggcaacaattaatagactggatggaggcggataaagttgcaggaccacttctgcgctcggcccttccggctggctggtttattgctgataaatctggagccggtgagcgtgggtctcgcggtatcattgcagcactggggccagatggtaagccctcccgtatcgtagttatctacacgacggggagtcaggcaactatggatgaacgaaatagacagatcgctgagataggtgcctcactgattaagcattggtaactgtcagaccaagtttactcatatatactttagattgatttaaaacttcatttttaatttaaaaggatctaggtgaagatcctttttgataatctcatgaccaaaatcccttaacgtgagttttcgttccactgagcgtcagaccccgtagaaaagatcaaaggatcttcttgagatcctttttttctgcgcgtaatctgctgcttgcaaacaaaaaaaccaccgctaccagcggtggtttgtttgccggatcaagagctaccaactctttttccgaaggtaactggcttcagcagagcgcagataccaaatactgttcttctagtgtagccgtagttaggccaccacttcaagaactctgtagcaccgcctacatacctcgctctgctaatcctgttaccagtggctgctgccagtggcgataagtcgtgtcttaccgggttggactcaagacgatagttaccggataaggcgcagcggtcgggctgaacggggggttcgtgcacacagcccagcttggagcgaacgacctacaccgaactgagatacctacagcgtgagctatgagaaagcgccacgcttcccgaagggagaaaggcggacaggtatccggtaagcggcagggtcggaacaggagagcgcacgagggagcttccagggggaaacgcctggtatctttatagtcctgtcgggtttcgccacctctgacttgagcgtcgatttttgtgatgctcgtcaggggggcggagcctatggaaaaacgccagcaacgcggcctttttacggttcctggccttttgctggccttttgctcacatgttctttcctgcgttatcccctgattctgtggataaccgtattaccgcctttgagtgagctgataccgctcgccgcagccgaacgaccgagcgcagcgagtcagtgagcgaggaagcggaagagcgcccaatacgcaaaccgcctctccccgcgcgttggccgattcattaatgcagctggcacgacaggtttcccgactggaaagcgggcagtgagcgcaacgcaattaatgtgagttagctcactcattaggcaccccaggctttacactttatgcttccggctcgtatgttgtgtggaattgtgagcggataacaatttcacacaggaaacagctatgaccatgattacgccaagcgcgcaattaaccctcactaaagggaacaaaagctggagctgcaagcttggccattgcatacgttgtatccatatcataatatgtacatttatattggctcatgtccaacattaccgccatgttgacattgattattgactagttattaatagtaatcaattacggggtcattagttcatagcccatatatggagttccgcgttacataacttacggtaaatggcccgcctggctgaccgcccaacgacccccgcccattgacgtcaataatgacgtatgttcccatagtaacgccaatagggactttccattgacgtcaatgggtggagtatttacggtaaactgcccacttggcagtacatcaagtgtatcatatgccaagtacgccccctattgacgtcaatgacggtaaatggcccgcctggcattatgcccagtacatgaccttatgggactttcctacttggcagtacatctacgtattagtcatcgctattaccatggtgatgcggttttggcagtacatcaatgggcgtggatagcggtttgactcacggggatttccaagtctccaccccattgacgtcaatgggagtttgttttggcaccaaaatcaacgggactttccaaaatgtcgtaacaactccgccccattgacgcaaatgggcggtaggcgtgtacggtgggaggtctatataagcagagctcgtttagtgaaccggggtctctctggttagaccagatctgagcctgggagctctctggctaactagggaacccactgcttaagcctcaataaagcttgccttgagtgcttcaagtagtgtgtgcccgtctgttgtgtgactctggtaactagagatccctcagacccttttagtcagtgtggaaaatctctagcagtggcgcccgaacagggacttgaaagcgaaagggaaaccagaggagctctctcgacgcaggactcggcttgctgaagcgcgcacggcaagaggcgaggggcggcgactggtgagtacgccaaaaattttgactagcggaggctagaaggagagagatgggtgcgagagcgtcagtattaagcgggggagaattagatcgcgatgggaaaaaattcggttaaggccagggggaaagaaaaaatataaattaaaacatatagtatgggcaagcagggagctagaacgattcgcagttaatcctggcctgttagaaacatcagaaggctgtagacaaatactgggacagctacaaccatcccttcagacaggatcagaagaacttagatcattatataatacagtagcaaccctctattgtgtgcatcaaaggatagagataaaagacaccaaggaagctttagacaagatagaggaagagcaaaacaaaagtaagaccaccgcacagcaagcggccgctgatcttcagacctggaggaggagatatgagggacaattggagaagtgaattatataaatataaagtagtaaaaattgaaccattaggagtagcacccaccaaggcaaagagaagagtggtgcagagagaaaaaagagcagtgggaataggagctttgttccttgggttcttgggagcagcaggaagcactatgggcgcagcctcaatgacgctgacggtacaggccagacaattattgtctggtatagtgcagcagcagaacaatttgctgagggctattgaggcgcaacagcatctgttgcaactcacagtctggggcatcaagcagctccaggcaagaatcctggctgtggaaagatacctaaaggatcaacagctcctggggatttggggttgctctggaaaactcatttgcaccactgctgtgccttggaatgctagttggagtaataaatctctggaacagatttggaatcacacgacctggatggagtgggacagagaaattaacaattacacaagcttaatacactccttaattgaagaatcgcaaaaccagcaagaaaagaatgaacaagaattattggaattagataaatgggcaagtttgtggaattggtttaacataacaaattggctgtggtatataaaattattcataatgatagtaggaggcttggtaggtttaagaatagtttttgctgtactttctatagtgaatagagttaggcagggatattcaccattatcgtttcagacccacctcccaaccccgaggggacccgacaggcccgaaggaatagaagaagaaggtggagagagagacagagacagatccattcgattagtgaacggatctcgacggtatcggttaacttttaaaagaaaaggggggattggggggtacagtgcaggggaaagaatagtagacataatagcaacagacatacaaactaaagaattacaaaaacaaattacaaaaattcaaaattttatcgatcacgagactagcctcgaggggaatttccggggactttccgggaatttccggggactttccgggaatttccgggaatttccggggactttccgggaatttccggggactttccgggaatttccctgcaggagactctagagggtatataatggtttaaacttaagcttggtaccgggcccccgaagacgcgtgccaccatggtgagcaagggcgaggagctgttcaccggggtggtgcccatcctggtcgagctggacggcgacgtaaacggccacaagttcagcgtgtccggcgagggcgagggcgatgccacctacggcaagctgaccctgaagttcatctgcaccaccggcaagctgcccgtgccctggcccaccctcgtgaccaccctgacctacggcgtgcagtgcttcagccgctaccccgaccacatgaagcagcacgacttcttcaagtccgccatgcccgaaggctacgtccaggagcgcaccatcttcttcaaggacgacggcaactacaagacccgcgccgaggtgaagttcgagggcgacaccctggtgaaccgcatcgagctgaagggcatcgacttcaaggaggacggcaacatcctggggcacaagctggagtacaactacaacagccacaacgtctatatcatggccgacaagcagaagaacggcatcaaggtgaacttcaagatccgccacaacatcgaggacggcagcgtgcagctcgccgaccactaccagcagaacacccccatcggcgacggccccgtgctgctgcccgacaaccactacctgagcacccagtccgccctgagcaaagaccccaacgagaagcgcgatcacatggtcctgctggagttcgtgaccgccgccgggatcactctcggcatggacgagctgtacaagtaatcgaattcccacggggttggggttgcgccttttccaaggcagccctgggtttgcgcagggacgcggctgctctgggcgtggttccgggaaacgcagcggcgccgaccctgggtctcgcacattcttcacgtccgttcgcagcgtcacccggatcttcgccgctacccttgtgggccccccggcgacgcttcctgctccgcccctaagtcgggaaggttccttgcggttcgcggcgtgccggacgtgacaaacggaagccgcacgtctcactagtaccctcgcagacggacagcgccagggagcaatggcagcgcgccgaccgcgatgggctgtggccaatagcggctgctcagcggggcgcgccgagagcagcggccgggaaggggcggtgcgggaggcggggtgtggggcggtagtgtgggccctgttcctgcccgcgcggtgttccgcattctgcaagcctccggagcgcacgtcggcagtcggctccctcgttgaccgaatcaccgacctctctccccagggggatccaccggtcacgtggctagcgccaccnnnnnnnnnnnnnnnnnnnnnnnnnnnnnnnnnnnnnnnnnnnnnnnnnnnnnnnnnnnnnnnnnnnnnnnnnnnnnnnnnnnnnnnnnnnnnnnnnnnnnnnnnnnnnnnnnnnnnnnnnnnnnnnnnnnnnnnnnnnnnnnnnnnnnnnnnnnnnnnnnnnnnnnnnnnnnnnnnnnnnnnnnnnnnnnnnnnnnnnnnnnnnnnnnnnnnnnnnnnnnnnnnnnnnnnnnnnnnnnnnnnnnnnnnnnnnnnnnnnnnnnnnnnnnnnnnnnnnnnnnnnnnnnnnnnnnnnnnnnnnnnnnnnnnnnnnnnnnnnnnnnnnnnnnnnnnnnnnnnnnnnnnnnnnnnnnnnnnnnnnnnnnnnnnnnnnnnnnnnnnnnnnnnnnnnnnnnnnnnnnnnnnnnnnnnnnnnnnnnnnnnnnnnnnnnnnnnnnnnnnnnnnnnnnnnnnnnnnnnnnnnnnnnnnnnnnnnnnnnnnnnnnnnnnnnnnnnnnnnnnnnnnnnnnnnnnnnnnnnnnnnnnnnnnnnnnnnnnnnnnnnnnnnnnnnnnnnnnnnnnnnnnnnnnnnnnnnnnnnnnnnnnnnnnnnnnnnnnnnnnnnnnnnnnnnnnnnnnnnnnnnnnnnnnnnnnnnnnnnnnnnnnnnnnnnnnnnnnnnnnnnnnnnnnnnnnnnnnnnnnnnnnnnnnnnnnnnnnnnnnnnnnnnnnnnnnnnnnnnnnnnnnnnnnnnnnnnnnnnnnnnnnnnnnnnnnnnnnnnnnnnnnnnnnnnnnnnnnnnnnnnnnnnnnnnnnnnnnnnnnnnnnnnnnnnnnnnnnnnnnnnnnnnnnnnnnnnnnnnnnnnnnnnnnnnnnnnnnnnnnnnnnnnnnnnnnnnnnnnnnnnnnnnnnnnnnnnnnnnnnnnnnnnnnnnnnnnnnnnnnnnnnnnnnnnnnnnnnnnnnnnnnnnnnnnnnnnnnnnnnnnnnnnnnnnnnnnnnnnnnnnnnnnnnnnnnnnnnnnnnnnnnnnnnnnnnnnnnnnnnnnnnnnnnnnnnnnnnnnnnnnnnnnnnnnnnnnnnnnnnnnnnnnnnnnnnnnnnnnnnnnnnnnnnnnnnnnnnnnnnnnnnnnnnnnnnnnnnnnnnnnnnnnnnnnnnnnnnnnnnnnnnnnnnnnnnnnnnnnnnnnnnnnnnnnnnnnnnnnnnnnnnnnnnnnnnnnnnnnnnnnnnnnnnnnnnnnnnnnnnnnnnnnnnnnnnnnnnnnnnnnnnnnnnnnnnnnnnnnnnnnnnnnnnnnnnnnnnnnnnnnnnnnnnnnnnnnnnnnnnnnnnnnnnnnnnnnnnnnnnnnnnnnnnnnnnnnnnnnnnnnnnnnnnnnnnnnnnnnnnnnnnnnnnnnnnnnnnnnnnnnnnnnnnnnnnnnnnnnnnnnnnnnnnnnnnnnnnnnnnnnnnnnnnnnnnnnnnnnnnnnnnnnnnnnnnnntaggatccgccggcggccgcgtcgacaatcaacctctggattacaaaatttgtgaaagattgactggtattcttaactatgttgctccttttacgctatgtggatacgctgctttaatgcctttgtatcatgctattgcttcccgtatggctttcattttctcctccttgtataaatcctggttgctgtctctttatgaggagttgtggcccgttgtcaggcaacgtggcgtggtgtgcactgtgtttgctgacgcaacccccactggttggggcattgccaccacctgtcagctcctttccgggactttcgctttccccctccctattgccacggcggaactcatcgccgcctgccttgcccgctgctggacaggggctcggctgttgggcactgacaattccgtggtgttgtcggggaagctgacgtcctttccatggctgctcgcctgtgttgccacctggattctgcgcgggacgtccttctgctacgtcccttcggccctcaatccagcggaccttccttcccgcggcctgctgccggctctgcggcctcttccgcgtcttcgccttcgccctcagacgagtcggatctccctttgggccgcctccccgcctggaattcgagctcggtacctttaagaccaatgacttacaaggcagctgtagatcttagccactttttaaaagaaaaggggggactggaagggctaattcactcccaacgaagacaagatctgctttttgcttgtactgggtctctctggttagaccagatctgagcctgggagctctctggctaactagggaacccactgcttaagcctcaataaagcttgccttgagtgcttcaagtagtgtgtgcccgtctgttgtgtgactctggtaactagagatccctcagacccttttagtcagtgtggaaaatctctagcagtagtagttcatgtcatcttattattcagtatttataacttgcaaagaaatgaatatcagagagtgagaggaacttgtttattgcagcttataatggttacaaataaagcaatagcatcacaaatttcacaaataaagcatttttttcactgcattctagttgtggtttgtccaaactcatcaatgtatcttatcatgtctggctctagctatcccgcccctaactccgcccagttccgcccattctccgccccatggctgactaattttttttatttatgcagaggccgaggccgcctcggcctctgagctattccagaagtagtgaggaggcttttttggaggcctaggcttttgcgtcgagacgtacccaattcgccctatagtgagtcgtattacgcgcgctcactggccgtcgttttacaacgtcgtgactgggaaaaccctggcgttacccaacttaatcgccttgcagcacatccccctttcgccagctggcgtaatagcgaagaggcccgcaccgatcgcccttcccaacagttgcgcagcctgaatggcgaatggcgcgacgcgccctgtagcggcgcattaagcgcggcgggtgtggtggttacgcgcagcgtgaccgctacacttgccagcgccctagcgcccgctcctttcgctttcttcccttcctttctcgccacgttcgccggctttccccgtcaagctctaaatcgggggctccctttagggttccgatttagtgctttacggcacctcgaccccaaaaaacttgattagggtgatggttcacgtagtgggccatcgccctgatagacggtttttcgccctttgacgttggagtccacgttctttaatagtggactcttgttccaaactggaacaacactcaaccctatctcggtctattcttttgatttataagggattttgccgatttcggcctattggttaaaaaatgagctgatttaacaaaaatttaacgcgaattttaacaaaatattaacgtttacaatttcccaggtggcacttttcggggaaatgtgcgcggaacccctatttgtttatttttctaaatacattcaaatatgtatccgctcatgagacaataaccctgataaatgcttcaataatattgaaaaaggaagagtatgagtattcaacatttccgtgtcgcccttattcccttttttgcggcattttgccttcctgtttttgctcacccagaaacgctggtgaaagtaaaagatgctgaagatcagttgggtgcacgagtgggttacatcgaactggatctcaacagcggtaagatccttgagagttttcgccccgaagaacgttttccaatgatgagcacttttaaagttctgctatgtggcgcggtattatcccgtattgacgccgggcaagagcaactcggtcgccgcatacactattctcagaatgacttggttg

SEQ ID NO: 25 - protein, 239 aa, Artificial Sequence; identical to SEQ ID NO: 9
  [CDS]:4351..5070 from SEQ ID NO 24

SEQ ID NO: 26 - DNA, 7705 bp, Artificial Sequence
  pCAS.NFATenhsyn.EGFP.PGK.CAR.PRE SIN
  promoter 446..1116: /note="CMV promoter"
  misc_feature 1117..1137: /note="part of R element"
  misc_feature 1138..1217: /note="U5 element"
  misc_feature 1218..1236: /note="PBS"
  promoter 1504..1747: /note="promoter NFATenhsyn"
  CDS 1760..2479: /gene="eGFP" /transl_table=1
  gene 3035..4489: /note="CAR"
  misc_feature 4732..5135: /note="WPRE: woodchuck hepatitis virus posttranscriptional regulatory element"
  misc_feature 5220..5273: /note="dU3 element"
  misc_feature 5274..5294: /note="part of R element"
ctgcctcgcgcgtttcggtgatgacggtgaaaacctctgacacatgcagctcccggagacggtcacagcttgtctgtaagcggatgccgggagcagacaagcccgtcagggcgcgtcagcgggtgttggcgggtgtcggggcgcagccatgacccagtcacgtagcgatagttactatgcggcatcagagcagattgtactgagagtgcaccatatgcggtgtgaaataccgcacagatgcgtaaggagaaaataccgcatcaggcgccattcgccattcaggctgcgcaactgttgggaagggcgatcggtgcgggcctcttcgctattacgccagctggcgaaagggggatgtgctgcaaggcgattaagttgggtaacgccagggttttcccagtcacgacgttgtaaaacgacggccagtgaattagtactctagcttaagccattgcatacgttgtatccatatcataatatgtacatttatattggctcatgtccaacattaccgccatgttgacattgattattgactagttattaatagtaatcaattacggggtcattagttcatagcccatatatggagttccgcgttacataacttacggtaaatggcccgcctggctgaccgcccaacgacccccgcccattgacgtcaataatgacgtatgttcccatagtaacgccaatagggactttccattgacgtcaatgggtggagtatttacggtaaactgcccacttggcagtacatcaagtgtatcatatgccaagtacgccccctattgacgtcaatgacggtaaatggcccgcctggcattatgcccagtacatgaccttatgggactttcctacttggcagtacatctacgtattagtcatcgctattaccatggtgatgcggttttggcagtacatcaatgggcgtggatagcggtttgactcacggggatttccaagtctccaccccattgacgtcaatgggagtttgttttggcaccaaaatcaacgggactttccaaaatgtcgtaacaactccgccccattgacgcaaatgggcggtaggcgtgtacggtgggaggtctatataagcagagctcgtttagtgaaccggccatttgaccattcaccacattggtgtgcacctgggttgatggccggaccgttgattccctgacgactacgagcacctgcatgaagcagaaggcttcatttggtgaccccgacgtgatagttagggaatagtggtcggccacagacggcgtggcgatcctgtctccatccgtctcgtctatcgggaggcgagttcgatgaccctggtggagggggctgcggcttagggaggcagaagctgagtaccgtcggagggagctccagggcccggagcgactgacccctgccgagaactcagagggtcgtcggaagacggagagtgagcccgacgaccaccccaggcacgtctttggtcggcctgcggatcaagcagggcccgctcgagcgtggaggaaaaactgtttcatacagaaggcgtggaggaaaaactgtttcatacagaaggcgtggaggaaaaactgtttcatacagaaggcgtggaggaaaaactgtttcatacagaaggcgtggaggaaaaactgtttcatacagaaggcgtggaggaaaaactgtttcatacagaaggcgtctgcaggagactctagagggtatataatggtttaaacttaagcttggtaccgggcccccgaagacgcgtgccaccatggtgagcaagggcgaggagctgttcaccggggtggtgcccatcctggtcgagctggacggcgacgtaaacggccacaagttcagcgtgtccggcgagggcgagggcgatgccacctacggcaagctgaccctgaagttcatctgcaccaccggcaagctgcccgtgccctggcccaccctcgtgaccaccctgacctacggcgtgcagtgcttcagccgctaccccgaccacatgaagcagcacgacttcttcaagtccgccatgcccgaaggctacgtccaggagcgcaccatcttcttcaaggacgacggcaactacaagacccgcgccgaggtgaagttcgagggcgacaccctggtgaaccgcatcgagctgaagggcatcgacttcaaggaggacggcaacatcctggggcacaagctggagtacaactacaacagccacaacgtctatatcatggccgacaagcagaagaacggcatcaaggtgaacttcaagatccgccacaacatcgaggacggcagcgtgcagctcgccgaccactaccagcagaacacccccatcggcgacggccccgtgctgctgcccgacaaccactacctgagcacccagtccgccctgagcaaagaccccaacgagaagcgcgatcacatggtcctgctggagttcgtgaccgccgccgggatcactctcggcatggacgagctgtacaagtaatcgaattcccacggggttggggttgcgccttttccaaggcagccctgggtttgcgcagggacgcggctgctctgggcgtggttccgggaaacgcagcggcgccgaccctgggtctcgcacattcttcacgtccgttcgcagcgtcacccggatcttcgccgctacccttgtgggccccccggcgacgcttcctgctccgcccctaagtcgggaaggttccttgcggttcgcggcgtgccggacgtgacaaacggaagccgcacgtctcactagtaccctcgcagacggacagcgccagggagcaatggcagcgcgccgaccgcgatgggctgtggccaatagcggctgctcagcggggcgcgccgagagcagcggccgggaaggggcggtgcgggaggcggggtgtggggcggtagtgtgggccctgttcctgcccgcgcggtgttccgcattctgcaagcctccggagcgcacgtcggcagtcggctccctcgttgaccgaatcaccgacctctctccccagggggatccaccggtcacgtggctagcgccaccnnnnnnnnnnnnnnnnnnnnnnnnnnnnnnnnnnnnnnnnnnnnnnnnnnnnnnnnnnnnnnnnnnnnnnnnnnnnnnnnnnnnnnnnnnnnnnnnnnnnnnnnnnnnnnnnnnnnnnnnnnnnnnnnnnnnnnnnnnnnnnnnnnnnnnnnnnnnnnnnnnnnnnnnnnnnnnnnnnnnnnnnnnnnnnnnnnnnnnnnnnnnnnnnnnnnnnnnnnnnnnnnnnnnnnnnnnnnnnnnnnnnnnnnnnnnnnnnnnnnnnnnnnnnnnnnnnnnnnnnnnnnnnnnnnnnnnnnnnnnnnnnnnnnnnnnnnnnnnnnnnnnnnnnnnnnnnnnnnnnnnnnnnnnnnnnnnnnnnnnnnnnnnnnnnnnnnnnnnnnnnnnnnnnnnnnnnnnnnnnnnnnnnnnnnnnnnnnnnnnnnnnnnnnnnnnnnnnnnnnnnnnnnnnnnnnnnnnnnnnnnnnnnnnnnnnnnnnnnnnnnnnnnnnnnnnnnnnnnnnnnnnnnnnnnnnnnnnnnnnnnnnnnnnnnnnnnnnnnnnnnnnnnnnnnnnnnnnnnnnnnnnnnnnnnnnnnnnnnnnnnnnnnnnnnnnnnnnnnnnnnnnnnnnnnnnnnnnnnnnnnnnnnnnnnnnnnnnnnnnnnnnnnnnnnnnnnnnnnnnnnnnnnnnnnnnnnnnnnnnnnnnnnnnnnnnnnnnnnnnnnnnnnnnnnnnnnnnnnnnnnnnnnnnnnnnnnnnnnnnnnnnnnnnnnnnnnnnnnnnnnnnnnnnnnnnnnnnnnnnnnnnnnnnnnnnnnnnnnnnnnnnnnnnnnnnnnnnnnnnnnnnnnnnnnnnnnnnnnnnnnnnnnnnnnnnnnnnnnnnnnnnnnnnnnnnnnnnnnnnnnnnnnnnnnnnnnnnnnnnnnnnnnnnnnnnnnnnnnnnnnnnnnnnnnnnnnnnnnnnnnnnnnnnnnnnnnnnnnnnnnnnnnnnnnnnnnnnnnnnnnnnnnnnnnnnnnnnnnnnnnnnnnnnnnnnnnnnnnnnnnnnnnnnnnnnnnnnnnnnnnnnnnnnnnnnnnnnnnnnnnnnnnnnnnnnnnnnnnnnnnnnnnnnnnnnnnnnnnnnnnnnnnnnnnnnnnnnnnnnnnnnnnnnnnnnnnnnnnnnnnnnnnnnnnnnnnnnnnnnnnnnnnnnnnnnnnnnnnnnnnnnnnnnnnnnnnnnnnnnnnnnnnnnnnnnnnnnnnnnnnnnnnnnnnnnnnnnnnnnnnnnnnnnnnnnnnnnnnnnnnnnnnnnnnnnnnnnnnnnnnnnnnnnnnnnnnnnnnnnnnnnnnnnnnnnnnnnnnnnnnnnnnnnnnnnnnnnnnnnnnnnnnnnnnnnnnnnnnnnnnnnnnnnnnnnnnnnnnnnnnnnnnnnnnnnnnnnnnnnnnnnnnnnnnnnnnnnnnnnnnnnnnnnnnnnnnnnnnnnnnnnnnnnnnnnnnntaggatccgccggcggccgcgtcgacggatcccccgggctgcaggaattcgagcatcttaccgccatttatacccatatttgttctgtttttcttgatttgggtatacatttaaatgttaataaaacaaaatggtggggcaatcatttacatttttagggatatgtaattactagttcaggtgtattgccacaagacaaacatgttaagaaactttcccgttatttacgctctgttcctgttaatcaacctctggattacaaaatttgtgaaagattgactgatattcttaactatgttgctccttttacgctgtgtggatatgctgctttaatgcctctgtatcatgctattgcttcccgtacggctttcgttttctcctccttgtataaatcctggttgctgtctctttatgaggagttgtggcccgttgtccgtcaacgtggcgtggtgtgctctgtgtttgctgacgcaacccccactggctggggcattgccaccacctgtcaactcctttctgggactttcgctttccccctcccgatcgccacggcagaactcatcgccgcctgccttgcccgctgctggacaggggctaggttgctgggcactgataattccgtggtgttgtcggggaagctgacgtcctttcgaattcgaaagcttttaaatatcgatgcgatgtacgggccagatatacgcgtatctgaggggactagggtgtgtttaggcgaaaagcggggcttcggttgtacgcggttaggagtccccttaggatatagtagtttcgcttttgcatagggagggggaaatgtagtcttatgcaatactcttgtacgtagtgcctagctcgatacaataaacgccatttgaccattcaccacattggtgtgcacctgggttgatggccggaccgttgattccctgacgactacgagcacctgcatgaagcagaaggcttcattctcgagagctttggcgtaatcatggtcatagctgtttcctgtgtgaaattgttatccgctcacaattccacacaacatacgagccggaagcataaagtgtaaagcctggggtgcctaatgagtgagctaactcacattaattgcgttgcgctcactgcccgctttccagtcgggaaacctgtcgtgccagctgcattaatgaatcggccaacgcgcggggagaggcggtttgcgtattgggcgctcttccgcttcctcgctcactgactcgctgcgctcggtcgttcggctgcggcgagcggtatcagctcactcaaaggcggtaatacggttatccacagaatcaggggataacgcaggaaagaacatgtgagcaaaaggccagcaaaaggccaggaaccgtaaaaaggccgcgttgctggcgtttttccataggctccgcccccctgacgagcatcacaaaaatcgacgctcaagtcagaggtggcgaaacccgacaggactataaagataccaggcgtttccccctggaagctccctcgtgcgctctcctgttccgaccctgccgcttaccggatacctgtccgcctttctcccttcgggaagcgtggcgctttctcaatgctcacgctgtaggtatctcagttcggtgtaggtcgttcgctccaagctgggctgtgtgcacgaaccccccgttcagcccgaccgctgcgccttatccggtaactatcgtcttgagtccaacccggtaagacacgacttatcgccactggcagcagccactggtaacaggattagcagagcgaggtatgtaggcggtgctacagagttcttgaagtggtggcctaactacggctacactagaaggacagtatttggtatctgcgctctgctgaagccagttaccttcggaaaaagagttggtagctcttgatccggcaaacaaaccaccgctggtagcggtggtttttttgtttgcaagcagcagattacgcgcagaaaaaaaggatctcaagaagatcctttgatcttttctacggggtctgacgctcagtggaacgaaaactcacgttaagggattttggtcatgagattatcaaaaaggatcttcacctagatccttttaaattaaaaatgaagttttaaatcaatctaaagtatatatgagtaaacttggtctgacagttaccaatgcttaatcagtgaggcacctatctcagcgatctgtctatttcgttcatccatagttgcctgactccccgtcgtgtagataactacgatacgggagggcttaccatctggccccagtgctgcaatgataccgcgagacccacgctcaccggctccagatttatcagcaataaaccagccagccggaagggccgagcgcagaagtggtcctgcaactttatccgcctccatccagtctattaattgttgccgggaagctagagtaagtagttcgccagttaatagtttgcgcaacgttgttgccattgctgctggcatcgtggtgtcacgctcgtcgtttggtatggcttcattcagctccggttcccaacgatcaaggcgagttacatgatcccccatgttgtgcaaaaaagcggttagctccttcggtcctccgatcgttgtcagaagtaagttggccgcagtgttatcactcatggttatggcagcactgcataattctcttactgtcatgccatccgtaagatgcttttctgtgactggtgagtactcaaccaagtcattctgagaatagtgtatgcggcgaccgagttgctcttgcccggcgtcaatacgggataataccgcgccacatagcagaactttaaaagtgctcatcattggaaaacgttcttcggggcgaaaactctcaaggatcttaccgctgttgagatccagttcgatgtaacccactcgtgcacccaactgatcttcagcatcttttactttcaccagcgtttctgggtgagcaaaaacaggaaggcaaaatgccgcaaaaaagggaataagggcgacacggaaatgttgaatactcatactcttcctttttcaatattattgaagcatttatcagggttattgtctcatgagcggatacatatttgaatgtatttagaaaaataaacaaataggggttccgcgcacatttccccgaaaagtgccacctgacgtctaagaaaccattattatcatgacattaacctataaaaataggcgtatcacgaggccctttcgtcttcaag

SEQ ID NO: 27 - protein, 239 aa, Artificial Sequence; identical to SEQ ID NO: 9
  [CDS]:1760..2479 from SEQ ID NO 26

SEQ ID NO: 28 - DNA, 7626 bp, Artificial Sequence
  pCAS.NFκBenhsyn.EGFP.PGK.CAR.PRE SIN
  promoter 1496..1668: /note="promoter NFκBenhsyn"
  CDS 1681..2400: /gene="eGFP" /transl_table=1
  gene 2956..4410: /gene="CAR"
  misc_feature 4460..5062: /note="PRE"
  misc_feature 4653..5056: /note="WPRE: woodchuck hepatitis virus posttranscriptional regulatory element"
ctgcctcgcgcgtttcggtgatgacggtgaaaacctctgacacatgcagctcccggagacggtcacagcttgtctgtaagcggatgccgggagcagacaagcccgtcagggcgcgtcagcgggtgttggcgggtgtcggggcgcagccatgacccagtcacgtagcgatagttactatgcggcatcagagcagattgtactgagagtgcaccatatgcggtgtgaaataccgcacagatgcgtaaggagaaaataccgcatcaggcgccattcgccattcaggctgcgcaactgttgggaagggcgatcggtgcgggcctcttcgctattacgccagctggcgaaagggggatgtgctgcaaggcgattaagttgggtaacgccagggttttcccagtcacgacgttgtaaaacgacggccagtgaattagtactctagcttaagccattgcatacgttgtatccatatcataatatgtacatttatattggctcatgtccaacattaccgccatgttgacattgattattgactagttattaatagtaatcaattacggggtcattagttcatagcccatatatggagttccgcgttacataacttacggtaaatggcccgcctggctgaccgcccaacgacccccgcccattgacgtcaataatgacgtatgttcccatagtaacgccaatagggactttccattgacgtcaatgggtggagtatttacggtaaactgcccacttggcagtacatcaagtgtatcatatgccaagtacgccccctattgacgtcaatgacggtaaatggcccgcctggcattatgcccagtacatgaccttatgggactttcctacttggcagtacatctacgtattagtcatcgctattaccatggtgatgcggttttggcagtacatcaatgggcgtggatagcggtttgactcacggggatttccaagtctccaccccattgacgtcaatgggagtttgttttggcaccaaaatcaacgggactttccaaaatgtcgtaacaactccgccccattgacgcaaatgggcggtaggcgtgtacggtgggaggtctatataagcagagctcgtttagtgaaccggccatttgaccattcaccacattggtgtgcacctgggttgatggccggaccgttgattccctgacgactacgagcacctgcatgaagcagaaggcttcatttggtgaccccgacgtgatagttagggaatagtggtcggccacagacggcgtggcgatcctgtctccatccgtctcgtctatcgggaggcgagttcgatgaccctggtggagggggctgcggcttagggaggcagaagctgagtaccgtcggagggagctccagggcccggagcgactgacccctgccgagaactcagagggtcgtcggaagacggagagtgagcccgacgaccaccccaggcacgtctttggtcggcctgcggatcaagcagggcccgctcgaggggaatttccggggactttccgggaatttccggggactttccgggaatttccgggaatttccggggactttccgggaatttccggggactttccgggaatttccctgcaggagactctagagggtatataatggtttaaacttaagcttggtaccgggcccccgaagacgcgtgccaccatggtgagcaagggcgaggagctgttcaccggggtggtgcccatcctggtcgagctggacggcgacgtaaacggccacaagttcagcgtgtccggcgagggcgagggcgatgccacctacggcaagctgaccctgaagttcatctgcaccaccggcaagctgcccgtgccctggcccaccctcgtgaccaccctgacctacggcgtgcagtgcttcagccgctaccccgaccacatgaagcagcacgacttcttcaagtccgccatgcccgaaggctacgtccaggagcgcaccatcttcttcaaggacgacggcaactacaagacccgcgccgaggtgaagttcgagggcgacaccctggtgaaccgcatcgagctgaagggcatcgacttcaaggaggacggcaacatcctggggcacaagctggagtacaactacaacagccacaacgtctatatcatggccgacaagcagaagaacggcatcaaggtgaacttcaagatccgccacaacatcgaggacggcagcgtgcagctcgccgaccactaccagcagaacacccccatcggcgacggccccgtgctgctgcccgacaaccactacctgagcacccagtccgccctgagcaaagaccccaacgagaagcgcgatcacatggtcctgctggagttcgtgaccgccgccgggatcactctcggcatggacgagctgtacaagtaatcgaattcccacggggttggggttgcgccttttccaaggcagccctgggtttgcgcagggacgcggctgctctgggcgtggttccgggaaacgcagcggcgccgaccctgggtctcgcacattcttcacgtccgttcgcagcgtcacccggatcttcgccgctacccttgtgggccccccggcgacgcttcctgctccgcccctaagtcgggaaggttccttgcggttcgcggcgtgccggacgtgacaaacggaagccgcacgtctcactagtaccctcgcagacggacagcgccagggagcaatggcagcgcgccgaccgcgatgggctgtggccaatagcggctgctcagcggggcgcgccgagagcagcggccgggaaggggcggtgcgggaggcggggtgtggggcggtagtgtgggccctgttcctgcccgcgcggtgttccgcattctgcaagcctccggagcgcacgtcggcagtcggctccctcgttgaccgaatcaccgacctctctccccagggggatccaccggtcacgtggctagcgccaccnnnnnnnnnnnnnnnnnnnnnnnnnnnnnnnnnnnnnnnnnnnnnnnnnnnnnnnnnnnnnnnnnnnnnnnnnnnnnnnnnnnnnnnnnnnnnnnnnnnnnnnnnnnnnnnnnnnnnnnnnnnnnnnnnnnnnnnnnnnnnnnnnnnnnnnnnnnnnnnnnnnnnnnnnnnnnnnnnnnnnnnnnnnnnnnnnnnnnnnnnnnnnnnnnnnnnnnnnnnnnnnnnnnnnnnnnnnnnnnnnnnnnnnnnnnnnnnnnnnnnnnnnnnnnnnnnnnnnnnnnnnnnnnnnnnnnnnnnnnnnnnnnnnnnnnnnnnnnnnnnnnnnnnnnnnnnnnnnnnnnnnnnnnnnnnnnnnnnnnnnnnnnnnnnnnnnnnnnnnnnnnnnnnnnnnnnnnnnnnnnnnnnnnnnnnnnnnnnnnnnnnnnnnnnnnnnnnnnnnnnnnnnnnnnnnnnnnnnnnnnnnnnnnnnnnnnnnnnnnnnnnnnnnnnnnnnnnnnnnnnnnnnnnnnnnnnnnnnnnnnnnnnnnnnnnnnnnnnnnnnnnnnnnnnnnnnnnnnnnnnnnnnnnnnnnnnnnnnnnnnnnnnnnnnnnnnnnnnnnnnnnnnnnnnnnnnnnnnnnnnnnnnnnnnnnnnnnnnnnnnnnnnnnnnnnnnnnnnnnnnnnnnnnnnnnnnnnnnnnnnnnnnnnnnnnnnnnnnnnnnnnnnnnnnnnnnnnnnnnnnnnnnnnnnnnnnnnnnnnnnnnnnnnnnnnnnnnnnnnnnnnnnnnnnnnnnnnnnnnnnnnnnnnnnnnnnnnnnnnnnnnnnnnnnnnnnnnnnnnnnnnnnnnnnnnnnnnnnnnnnnnnnnnnnnnnnnnnnnnnnnnnnnnnnnnnnnnnnnnnnnnnnnnnnnnnnnnnnnnnnnnnnnnnnnnnnnnnnnnnnnnnnnnnnnnnnnnnnnnnnnnnnnnnnnnnnnnnnnnnnnnnnnnnnnnnnnnnnnnnnnnnnnnnnnnnnnnnnnnnnnnnnnnnnnnnnnnnnnnnnnnnnnnnnnnnnnnnnnnnnnnnnnnnnnnnnnnnnnnnnnnnnnnnnnnnnnnnnnnnnnnnnnnnnnnnnnnnnnnnnnnnnnnnnnnnnnnnnnnnnnnnnnnnnnnnnnnnnnnnnnnnnnnnnnnnnnnnnnnnnnnnnnnnnnnnnnnnnnnnnnnnnnnnnnnnnnnnnnnnnnnnnnnnnnnnnnnnnnnnnnnnnnnnnnnnnnnnnnnnnnnnnnnnnnnnnnnnnnnnnnnnnnnnnnnnnnnnnnnnnnnnnnnnnnnnnnnnnnnnnnnnnnnnnnnnnnnnnnnnnnnnnnnnnnnnnnnnnnnnnnnnnnnnnnnnnnnnnnnnnnnnnnnnnnnnnnnnnnnnnnnnnnnnnnnnnnnnnnnnnnnnnnnnnnnnnnnnnnnnnnnnnnnnnnnnnnnnnnnnnnnnnnnnnnnnnnntaggatccgccggcggccgcgtcgacggatcccccgggctgcaggaattcgagcatcttaccgccatttatacccatatttgttctgtttttcttgatttgggtatacatttaaatgttaataaaacaaaatggtggggcaatcatttacatttttagggatatgtaattactagttcaggtgtattgccacaagacaaacatgttaagaaactttcccgttatttacgctctgttcctgttaatcaacctctggattacaaaatttgtgaaagattgactgatattcttaactatgttgctccttttacgctgtgtggatatgctgctttaatgcctctgtatcatgctattgcttcccgtacggctttcgttttctcctccttgtataaatcctggttgctgtctctttatgaggagttgtggcccgttgtccgtcaacgtggcgtggtgtgctctgtgtttgctgacgcaacccccactggctggggcattgccaccacctgtcaactcctttctgggactttcgctttccccctcccgatcgccacggcagaactcatcgccgcctgccttgcccgctgctggacaggggctaggttgctgggcactgataattccgtggtgttgtcggggaagctgacgtcctttcgaattcgaaagcttttaaatatcgatgcgatgtacgggccagatatacgcgtatctgaggggactagggtgtgtttaggcgaaaagcggggcttcggttgtacgcggttaggagtccccttaggatatagtagtttcgcttttgcatagggagggggaaatgtagtcttatgcaatactcttgtacgtagtgcctagctcgatacaataaacgccatttgaccattcaccacattggtgtgcacctgggttgatggccggaccgttgattccctgacgactacgagcacctgcatgaagcagaaggcttcattctcgagagctttggcgtaatcatggtcatagctgtttcctgtgtgaaattgttatccgctcacaattccacacaacatacgagccggaagcataaagtgtaaagcctggggtgcctaatgagtgagctaactcacattaattgcgttgcgctcactgcccgctttccagtcgggaaacctgtcgtgccagctgcattaatgaatcggccaacgcgcggggagaggcggtttgcgtattgggcgctcttccgcttcctcgctcactgactcgctgcgctcggtcgttcggctgcggcgagcggtatcagctcactcaaaggcggtaatacggttatccacagaatcaggggataacgcaggaaagaacatgtgagcaaaaggccagcaaaaggccaggaaccgtaaaaaggccgcgttgctggcgtttttccataggctccgcccccctgacgagcatcacaaaaatcgacgctcaagtcagaggtggcgaaacccgacaggactataaagataccaggcgtttccccctggaagctccctcgtgcgctctcctgttccgaccctgccgcttaccggatacctgtccgcctttctcccttcgggaagcgtggcgctttctcaatgctcacgctgtaggtatctcagttcggtgtaggtcgttcgctccaagctgggctgtgtgcacgaaccccccgttcagcccgaccgctgcgccttatccggtaactatcgtcttgagtccaacccggtaagacacgacttatcgccactggcagcagccactggtaacaggattagcagagcgaggtatgtaggcggtgctacagagttcttgaagtggtggcctaactacggctacactagaaggacagtatttggtatctgcgctctgctgaagccagttaccttcggaaaaagagttggtagctcttgatccggcaaacaaaccaccgctggtagcggtggtttttttgtttgcaagcagcagattacgcgcagaaaaaaaggatctcaagaagatcctttgatcttttctacggggtctgacgctcagtggaacgaaaactcacgttaagggattttggtcatgagattatcaaaaaggatcttcacctagatccttttaaattaaaaatgaagttttaaatcaatctaaagtatatatgagtaaacttggtctgacagttaccaatgcttaatcagtgaggcacctatctcagcgatctgtctatttcgttcatccatagttgcctgactccccgtcgtgtagataactacgatacgggagggcttaccatctggccccagtgctgcaatgataccgcgagacccacgctcaccggctccagatttatcagcaataaaccagccagccggaagggccgagcgcagaagtggtcctgcaactttatccgcctccatccagtctattaattgttgccgggaagctagagtaagtagttcgccagttaatagtttgcgcaacgttgttgccattgctgctggcatcgtggtgtcacgctcgtcgtttggtatggcttcattcagctccggttcccaacgatcaaggcgagttacatgatcccccatgttgtgcaaaaaagcggttagctccttcggtcctccgatcgttgtcagaagtaagttggccgcagtgttatcactcatggttatggcagcactgcataattctcttactgtcatgccatccgtaagatgcttttctgtgactggtgagtactcaaccaagtcattctgagaatagtgtatgcggcgaccgagttgctcttgcccggcgtcaatacgggataataccgcgccacatagcagaactttaaaagtgctcatcattggaaaacgttcttcggggcgaaaactctcaaggatcttaccgctgttgagatccagttcgatgtaacccactcgtgcacccaactgatcttcagcatcttttactttcaccagcgtttctgggtgagcaaaaacaggaaggcaaaatgccgcaaaaaagggaataagggcgacacggaaatgttgaatactcatactcttcctttttcaatattattgaagcatttatcagggttattgtctcatgagcggatacatatttgaatgtatttagaaaaataaacaaataggggttccgcgcacatttccccgaaaagtgccacctgacgtctaagaaaccattattatcatgacattaacctataaaaataggcgtatcacgaggccctttcgtcttcaag

SEQ ID NO: 29 - protein, 239 aa, Artificial Sequence; identical to SEQ ID NO: 9
  [CDS]:1681..2400 from SEQ ID NO 28

SEQ ID NO: 30 - protein, 239 aa, Artificial Sequence; identical to SEQ ID NO: 9
  [CDS]:4430..5149 from SEQ ID NO 8

SEQ ID NO: 31 - DNA, 224 bp, Artificial Sequence
  NFκBmIL2 promoter
  TATA_signal 151..157: /note="TATA box"
gggaatttccggggactttccgggaatttccggggactttccgggaatttccgggaatttccggggactttccgggaatttccggggactttccgggaatttcccccgggacattttgacacccccataatatttttccagaattaacagtataaattgcatctcttgttcaagagttccctatcactctctttaatcactactcacagtaacctcaactcctg

SEQ ID NO: 32 - DNA, 9544 bp, Artificial Sequence
  pCCL.PPT.NFκBmIL2.EGFP.PGK.CAR.WPRE
  misc_signal 2683..2808: /note="HIV-1 psi packaging signal of human immunodeficiency virus type 1"
  misc_feature 3301..3535: /note="RRE - Rev response element of HIV-1 allows for Rev-dependent mRNA export from the nucleus to the cytoplasm"
  misc_feature 4030..4147: /note="cPPT/CTS: central polypurine tract and central termination sequence of HIV-1"
  promoter 4178..4281: /note="NFκB"
  promoter 4178..4400: /note="NFκBmIL2"
  misc_feature 4282..4400: /note="mIL2"
  CDS 4419..5138: /gene="eGFP" /transl_table=1
  misc_feature 5694..7148: /note="CAR"
  misc_feature 7163..7768: /note="PRE"
  misc_feature 7175..7763: /note="WPRE: woodchuck hepatitis virus posttranscriptional regulatory element"
agtactcaccagtcacagaaaagcatcttacggatggcatgacagtaagagaattatgcagtgctgccataaccatgagtgataacactgcggccaacttacttctgacaacgatcggaggaccgaaggagctaaccgcttttttgcacaacatgggggatcatgtaactcgccttgatcgttgggaaccggagctgaatgaagccataccaaacgacgagcgtgacaccacgatgcctgtagcaatggcaacaacgttgcgcaaactattaactggcgaactacttactctagcttcccggcaacaattaatagactggatggaggcggataaagttgcaggaccacttctgcgctcggcccttccggctggctggtttattgctgataaatctggagccggtgagcgtgggtctcgcggtatcattgcagcactggggccagatggtaagccctcccgtatcgtagttatctacacgacggggagtcaggcaactatggatgaacgaaatagacagatcgctgagataggtgcctcactgattaagcattggtaactgtcagaccaagtttactcatatatactttagattgatttaaaacttcatttttaatttaaaaggatctaggtgaagatcctttttgataatctcatgaccaaaatcccttaacgtgagttttcgttccactgagcgtcagaccccgtagaaaagatcaaaggatcttcttgagatcctttttttctgcgcgtaatctgctgcttgcaaacaaaaaaaccaccgctaccagcggtggtttgtttgccggatcaagagctaccaactctttttccgaaggtaactggcttcagcagagcgcagataccaaatactgttcttctagtgtagccgtagttaggccaccacttcaagaactctgtagcaccgcctacatacctcgctctgctaatcctgttaccagtggctgctgccagtggcgataagtcgtgtcttaccgggttggactcaagacgatagttaccggataaggcgcagcggtcgggctgaacggggggttcgtgcacacagcccagcttggagcgaacgacctacaccgaactgagatacctacagcgtgagctatgagaaagcgccacgcttcccgaagggagaaaggcggacaggtatccggtaagcggcagggtcggaacaggagagcgcacgagggagcttccagggggaaacgcctggtatctttatagtcctgtcgggtttcgccacctctgacttgagcgtcgatttttgtgatgctcgtcaggggggcggagcctatggaaaaacgccagcaacgcggcctttttacggttcctggccttttgctggccttttgctcacatgttctttcctgcgttatcccctgattctgtggataaccgtattaccgcctttgagtgagctgataccgctcgccgcagccgaacgaccgagcgcagcgagtcagtgagcgaggaagcggaagagcgcccaatacgcaaaccgcctctccccgcgcgttggccgattcattaatgcagctggcacgacaggtttcccgactggaaagcgggcagtgagcgcaacgcaattaatgtgagttagctcactcattaggcaccccaggctttacactttatgcttccggctcgtatgttgtgtggaattgtgagcggataacaatttcacacaggaaacagctatgaccatgattacgccaagcgcgcaattaaccctcactaaagggaacaaaagctggagctgcaagcttggccattgcatacgttgtatccatatcataatatgtacatttatattggctcatgtccaacattaccgccatgttgacattgattattgactagttattaatagtaatcaattacggggtcattagttcatagcccatatatggagttccgcgttacataacttacggtaaatggcccgcctggctgaccgcccaacgacccccgcccattgacgtcaataatgacgtatgttcccatagtaacgccaatagggactttccattgacgtcaatgggtggagtatttacggtaaactgcccacttggcagtacatcaagtgtatcatatgccaagtacgccccctattgacgtcaatgacggtaaatggcccgcctggcattatgcccagtacatgaccttatgggactttcctacttggcagtacatctacgtattagtcatcgctattaccatggtgatgcggttttggcagtacatcaatgggcgtggatagcggtttgactcacggggatttccaagtctccaccccattgacgtcaatgggagtttgttttggcaccaaaatcaacgggactttccaaaatgtcgtaacaactccgccccattgacgcaaatgggcggtaggcgtgtacggtgggaggtctatataagcagagctcgtttagtgaaccggggtctctctggttagaccagatctgagcctgggagctctctggctaactagggaacccactgcttaagcctcaataaagcttgccttgagtgcttcaagtagtgtgtgcccgtctgttgtgtgactctggtaactagagatccctcagacccttttagtcagtgtggaaaatctctagcagtggcgcccgaacagggacttgaaagcgaaagggaaaccagaggagctctctcgacgcaggactcggcttgctgaagcgcgcacggcaagaggcgaggggcggcgactggtgagtacgccaaaaattttgactagcggaggctagaaggagagagatgggtgcgagagcgtcagtattaagcgggggagaattagatcgcgatgggaaaaaattcggttaaggccagggggaaagaaaaaatataaattaaaacatatagtatgggcaagcagggagctagaacgattcgcagttaatcctggcctgttagaaacatcagaaggctgtagacaaatactgggacagctacaaccatcccttcagacaggatcagaagaacttagatcattatataatacagtagcaaccctctattgtgtgcatcaaaggatagagataaaagacaccaaggaagctttagacaagatagaggaagagcaaaacaaaagtaagaccaccgcacagcaagcggccgctgatcttcagacctggaggaggagatatgagggacaattggagaagtgaattatataaatataaagtagtaaaaattgaaccattaggagtagcacccaccaaggcaaagagaagagtggtgcagagagaaaaaagagcagtgggaataggagctttgttccttgggttcttgggagcagcaggaagcactatgggcgcagcctcaatgacgctgacggtacaggccagacaattattgtctggtatagtgcagcagcagaacaatttgctgagggctattgaggcgcaacagcatctgttgcaactcacagtctggggcatcaagcagctccaggcaagaatcctggctgtggaaagatacctaaaggatcaacagctcctggggatttggggttgctctggaaaactcatttgcaccactgctgtgccttggaatgctagttggagtaataaatctctggaacagatttggaatcacacgacctggatggagtgggacagagaaattaacaattacacaagcttaatacactccttaattgaagaatcgcaaaaccagcaagaaaagaatgaacaagaattattggaattagataaatgggcaagtttgtggaattggtttaacataacaaattggctgtggtatataaaattattcataatgatagtaggaggcttggtaggtttaagaatagtttttgctgtactttctatagtgaatagagttaggcagggatattcaccattatcgtttcagacccacctcccaaccccgaggggacccgacaggcccgaaggaatagaagaagaaggtggagagagagacagagacagatccattcgattagtgaacggatctcgacggtatcggttaacttttaaaagaaaaggggggattggggggtacagtgcaggggaaagaatagtagacataatagcaacagacatacaaactaaagaattacaaaaacaaattacaaaaattcaaaattttatcgatcacgagactagcctcgacagcgctgggaatttccggggactttccgggaatttccggggactttccgggaatttccgggaatttccggggactttccgggaatttccggggactttccgggaatttcccccgggacattttgacacccccataatatttttccagaattaacagtataaattgcatctcttgttcaagagttccctatcactctctttaatcactactcacagtaacctcaactcctggatccacgcgtgccaccatggtgagcaagggcgaggagctgttcaccggggtggtgcccatcctggtcgagctggacggcgacgtaaacggccacaagttcagcgtgtccggcgagggcgagggcgatgccacctacggcaagctgaccctgaagttcatctgcaccaccggcaagctgcccgtgccctggcccaccctcgtgaccaccctgacctacggcgtgcagtgcttcagccgctaccccgaccacatgaagcagcacgacttcttcaagtccgccatgcccgaaggctacgtccaggagcgcaccatcttcttcaaggacgacggcaactacaagacccgcgccgaggtgaagttcgagggcgacaccctggtgaaccgcatcgagctgaagggcatcgacttcaaggaggacggcaacatcctggggcacaagctggagtacaactacaacagccacaacgtctatatcatggccgacaagcagaagaacggcatcaaggtgaacttcaagatccgccacaacatcgaggacggcagcgtgcagctcgccgaccactaccagcagaacacccccatcggcgacggccccgtgctgctgcccgacaaccactacctgagcacccagtccgccctgagcaaagaccccaacgagaagcgcgatcacatggtcctgctggagttcgtgaccgccgccgggatcactctcggcatggacgagctgtacaagtaatcgaattcccacggggttggggttgcgccttttccaaggcagccctgggtttgcgcagggacgcggctgctctgggcgtggttccgggaaacgcagcggcgccgaccctgggtctcgcacattcttcacgtccgttcgcagcgtcacccggatcttcgccgctacccttgtgggccccccggcgacgcttcctgctccgcccctaagtcgggaaggttccttgcggttcgcggcgtgccggacgtgacaaacggaagccgcacgtctcactagtaccctcgcagacggacagcgccagggagcaatggcagcgcgccgaccgcgatgggctgtggccaatagcggctgctcagcggggcgcgccgagagcagcggccgggaaggggcggtgcgggaggcggggtgtggggcggtagtgtgggccctgttcctgcccgcgcggtgttccgcattctgcaagcctccggagcgcacgtcggcagtcggctccctcgttgaccgaatcaccgacctctctccccagggggatccaccggtcacgtggctagcgccaccnnnnnnnnnnnnnnnnnnnnnnnnnnnnnnnnnnnnnnnnnnnnnnnnnnnnnnnnnnnnnnnnnnnnnnnnnnnnnnnnnnnnnnnnnnnnnnnnnnnnnnnnnnnnnnnnnnnnnnnnnnnnnnnnnnnnnnnnnnnnnnnnnnnnnnnnnnnnnnnnnnnnnnnnnnnnnnnnnnnnnnnnnnnnnnnnnnnnnnnnnnnnnnnnnnnnnnnnnnnnnnnnnnnnnnnnnnnnnnnnnnnnnnnnnnnnnnnnnnnnnnnnnnnnnnnnnnnnnnnnnnnnnnnnnnnnnnnnnnnnnnnnnnnnnnnnnnnnnnnnnnnnnnnnnnnnnnnnnnnnnnnnnnnnnnnnnnnnnnnnnnnnnnnnnnnnnnnnnnnnnnnnnnnnnnnnnnnnnnnnnnnnnnnnnnnnnnnnnnnnnnnnnnnnnnnnnnnnnnnnnnnnnnnnnnnnnnnnnnnnnnnnnnnnnnnnnnnnnnnnnnnnnnnnnnnnnnnnnnnnnnnnnnnnnnnnnnnnnnnnnnnnnnnnnnnnnnnnnnnnnnnnnnnnnnnnnnnnnnnnnnnnnnnnnnnnnnnnnnnnnnnnnnnnnnnnnnnnnnnnnnnnnnnnnnnnnnnnnnnnnnnnnnnnnnnnnnnnnnnnnnnnnnnnnnnnnnnnnnnnnnnnnnnnnnnnnnnnnnnnnnnnnnnnnnnnnnnnnnnnnnnnnnnnnnnnnnnnnnnnnnnnnnnnnnnnnnnnnnnnnnnnnnnnnnnnnnnnnnnnnnnnnnnnnnnnnnnnnnnnnnnnnnnnnnnnnnnnnnnnnnnnnnnnnnnnnnnnnnnnnnnnnnnnnnnnnnnnnnnnnnnnnnnnnnnnnnnnnnnnnnnnnnnnnnnnnnnnnnnnnnnnnnnnnnnnnnnnnnnnnnnnnnnnnnnnnnnnnnnnnnnnnnnnnnnnnnnnnnnnnnnnnnnnnnnnnnnnnnnnnnnnnnnnnnnnnnnnnnnnnnnnnnnnnnnnnnnnnnnnnnnnnnnnnnnnnnnnnnnnnnnnnnnnnnnnnnnnnnnnnnnnnnnnnnnnnnnnnnnnnnnnnnnnnnnnnnnnnnnnnnnnnnnnnnnnnnnnnnnnnnnnnnnnnnnnnnnnnnnnnnnnnnnnnnnnnnnnnnnnnnnnnnnnnnnnnnnnnnnnnnnnnnnnnnnnnnnnnnnnnnnnnnnnnnnnnnnnnnnnnnnnnnnnnnnnnnnnnnnnnnnnnnnnnnnnnnnnnnnnnnnnnnnnnnnnnnnnnnnnnnnnnnnnnnnnnnnnnnnnnnnnnnnnnnnnnnnnnnnnnnnnnnnnnnnnnnnnnnnnnnnnnnnnnnnnnnnnnnnnnnnnnnnnnnnnnnnnnnnnnnnnnnnnnnnnnnnnnnnnnnnnnnnnnnnnnnnnnnnnnnnnnnnnnnnnnnnnnnnnnnnnnnnnnnnnnnnnnnnnnnnnnnnnnnnnnnntaggatccgccggcggccgcgtcgacaatcaacctctggattacaaaatttgtgaaagattgactggtattcttaactatgttgctccttttacgctatgtggatacgctgctttaatgcctttgtatcatgctattgcttcccgtatggctttcattttctcctccttgtataaatcctggttgctgtctctttatgaggagttgtggcccgttgtcaggcaacgtggcgtggtgtgcactgtgtttgctgacgcaacccccactggttggggcattgccaccacctgtcagctcctttccgggactttcgctttccccctccctattgccacggcggaactcatcgccgcctgccttgcccgctgctggacaggggctcggctgttgggcactgacaattccgtggtgttgtcggggaagctgacgtcctttccatggctgctcgcctgtgttgccacctggattctgcgcgggacgtccttctgctacgtcccttcggccctcaatccagcggaccttccttcccgcggcctgctgccggctctgcggcctcttccgcgtcttcgccttcgccctcagacgagtcggatctccctttgggccgcctccccgcctggaattcgagctcggtacctttaagaccaatgacttacaaggcagctgtagatcttagccactttttaaaagaaaaggggggactggaagggctaattcactcccaacgaagacaagatctgctttttgcttgtactgggtctctctggttagaccagatctgagcctgggagctctctggctaactagggaacccactgcttaagcctcaataaagcttgccttgagtgcttcaagtagtgtgtgcccgtctgttgtgtgactctggtaactagagatccctcagacccttttagtcagtgtggaaaatctctagcagtagtagttcatgtcatcttattattcagtatttataacttgcaaagaaatgaatatcagagagtgagaggaacttgtttattgcagcttataatggttacaaataaagcaatagcatcacaaatttcacaaataaagcatttttttcactgcattctagttgtggtttgtccaaactcatcaatgtatcttatcatgtctggctctagctatcccgcccctaactccgcccagttccgcccattctccgccccatggctgactaattttttttatttatgcagaggccgaggccgcctcggcctctgagctattccagaagtagtgaggaggcttttttggaggcctaggcttttgcgtcgagacgtacccaattcgccctatagtgagtcgtattacgcgcgctcactggccgtcgttttacaacgtcgtgactgggaaaaccctggcgttacccaacttaatcgccttgcagcacatccccctttcgccagctggcgtaatagcgaagaggcccgcaccgatcgcccttcccaacagttgcgcagcctgaatggcgaatggcgcgacgcgccctgtagcggcgcattaagcgcggcgggtgtggtggttacgcgcagcgtgaccgctacacttgccagcgccctagcgcccgctcctttcgctttcttcccttcctttctcgccacgttcgccggctttccccgtcaagctctaaatcgggggctccctttagggttccgatttagtgctttacggcacctcgaccccaaaaaacttgattagggtgatggttcacgtagtgggccatcgccctgatagacggtttttcgccctttgacgttggagtccacgttctttaatagtggactcttgttccaaactggaacaacactcaaccctatctcggtctattcttttgatttataagggattttgccgatttcggcctattggttaaaaaatgagctgatttaacaaaaatttaacgcgaattttaacaaaatattaacgtttacaatttcccaggtggcacttttcggggaaatgtgcgcggaacccctatttgtttatttttctaaatacattcaaatatgtatccgctcatgagacaataaccctgataaatgcttcaataatattgaaaaaggaagagtatgagtattcaacatttccgtgtcgcccttattcccttttttgcggcattttgccttcctgtttttgctcacccagaaacgctggtgaaagtaaaagatgctgaagatcagttgggtgcacgagtgggttacatcgaactggatctcaacagcggtaagatccttgagagttttcgccccgaagaacgttttccaatgatgagcacttttaaagttctgctatgtggcgcggtattatcccgtattgacgccgggcaagagcaactcggtcgccgcatacactattctcagaatgacttggttg

SEQ ID NO: 33 - protein, 239 aa, Artificial Sequence; identical to SEQ ID NO: 9
  [CDS]:4419..5138 from SEQ ID NO 32

SEQ ID NO: 34 - DNA, 9314 bp, Artificial Sequence
  pCCL.PPT.NFATenhsyn.humanIL21co.PGK.CAR.PRE
  enhancer 1858..2237: /note="CMV enhancer"
  promoter 2238..2441: /note="CMV promoter"
  LTR 2456..2636: /note="5´LTR"
  misc_signal 2683..2808: /note="HIV-1 psi packaging signal"
  misc_signal 3301..3534: /note="RRE rev response element fo HIV-1, allows fo Rev-dependent mRNA export for nucleus to cytoplasm"
  misc_feature 4030..4147: /note="cPPT/CTS central purine tract and central termination sequence of HIV-1"
  promoter 4174..4417: /note="NFATenhsyn"
  gene 4430..4916: /gene="human IL21, codon-optimized"
  promoter 4921..5431: /note="hPGK promoter"
  gene 5464..6918: /note="placeholder for CAR"
  misc_signal 6945..7533: /note="WPRE"
  LTR 7620..8046: /note="3´LTR (delta U3), self-inactivating 3´ long terminal repeat (LTR) of HIV-1"
agtactcaccagtcacagaaaagcatcttacggatggcatgacagtaagagaattatgcagtgctgccataaccatgagtgataacactgcggccaacttacttctgacaacgatcggaggaccgaaggagctaaccgcttttttgcacaacatgggggatcatgtaactcgccttgatcgttgggaaccggagctgaatgaagccataccaaacgacgagcgtgacaccacgatgcctgtagcaatggcaacaacgttgcgcaaactattaactggcgaactacttactctagcttcccggcaacaattaatagactggatggaggcggataaagttgcaggaccacttctgcgctcggcccttccggctggctggtttattgctgataaatctggagccggtgagcgtgggtctcgcggtatcattgcagcactggggccagatggtaagccctcccgtatcgtagttatctacacgacggggagtcaggcaactatggatgaacgaaatagacagatcgctgagataggtgcctcactgattaagcattggtaactgtcagaccaagtttactcatatatactttagattgatttaaaacttcatttttaatttaaaaggatctaggtgaagatcctttttgataatctcatgaccaaaatcccttaacgtgagttttcgttccactgagcgtcagaccccgtagaaaagatcaaaggatcttcttgagatcctttttttctgcgcgtaatctgctgcttgcaaacaaaaaaaccaccgctaccagcggtggtttgtttgccggatcaagagctaccaactctttttccgaaggtaactggcttcagcagagcgcagataccaaatactgttcttctagtgtagccgtagttaggccaccacttcaagaactctgtagcaccgcctacatacctcgctctgctaatcctgttaccagtggctgctgccagtggcgataagtcgtgtcttaccgggttggactcaagacgatagttaccggataaggcgcagcggtcgggctgaacggggggttcgtgcacacagcccagcttggagcgaacgacctacaccgaactgagatacctacagcgtgagctatgagaaagcgccacgcttcccgaagggagaaaggcggacaggtatccggtaagcggcagggtcggaacaggagagcgcacgagggagcttccagggggaaacgcctggtatctttatagtcctgtcgggtttcgccacctctgacttgagcgtcgatttttgtgatgctcgtcaggggggcggagcctatggaaaaacgccagcaacgcggcctttttacggttcctggccttttgctggccttttgctcacatgttctttcctgcgttatcccctgattctgtggataaccgtattaccgcctttgagtgagctgataccgctcgccgcagccgaacgaccgagcgcagcgagtcagtgagcgaggaagcggaagagcgcccaatacgcaaaccgcctctccccgcgcgttggccgattcattaatgcagctggcacgacaggtttcccgactggaaagcgggcagtgagcgcaacgcaattaatgtgagttagctcactcattaggcaccccaggctttacactttatgcttccggctcgtatgttgtgtggaattgtgagcggataacaatttcacacaggaaacagctatgaccatgattacgccaagcgcgcaattaaccctcactaaagggaacaaaagctggagctgcaagcttggccattgcatacgttgtatccatatcataatatgtacatttatattggctcatgtccaacattaccgccatgttgacattgattattgactagttattaatagtaatcaattacggggtcattagttcatagcccatatatggagttccgcgttacataacttacggtaaatggcccgcctggctgaccgcccaacgacccccgcccattgacgtcaataatgacgtatgttcccatagtaacgccaatagggactttccattgacgtcaatgggtggagtatttacggtaaactgcccacttggcagtacatcaagtgtatcatatgccaagtacgccccctattgacgtcaatgacggtaaatggcccgcctggcattatgcccagtacatgaccttatgggactttcctacttggcagtacatctacgtattagtcatcgctattaccatggtgatgcggttttggcagtacatcaatgggcgtggatagcggtttgactcacggggatttccaagtctccaccccattgacgtcaatgggagtttgttttggcaccaaaatcaacgggactttccaaaatgtcgtaacaactccgccccattgacgcaaatgggcggtaggcgtgtacggtgggaggtctatataagcagagctcgtttagtgaaccggggtctctctggttagaccagatctgagcctgggagctctctggctaactagggaacccactgcttaagcctcaataaagcttgccttgagtgcttcaagtagtgtgtgcccgtctgttgtgtgactctggtaactagagatccctcagacccttttagtcagtgtggaaaatctctagcagtggcgcccgaacagggacttgaaagcgaaagggaaaccagaggagctctctcgacgcaggactcggcttgctgaagcgcgcacggcaagaggcgaggggcggcgactggtgagtacgccaaaaattttgactagcggaggctagaaggagagagatgggtgcgagagcgtcagtattaagcgggggagaattagatcgcgatgggaaaaaattcggttaaggccagggggaaagaaaaaatataaattaaaacatatagtatgggcaagcagggagctagaacgattcgcagttaatcctggcctgttagaaacatcagaaggctgtagacaaatactgggacagctacaaccatcccttcagacaggatcagaagaacttagatcattatataatacagtagcaaccctctattgtgtgcatcaaaggatagagataaaagacaccaaggaagctttagacaagatagaggaagagcaaaacaaaagtaagaccaccgcacagcaagcggccgctgatcttcagacctggaggaggagatatgagggacaattggagaagtgaattatataaatataaagtagtaaaaattgaaccattaggagtagcacccaccaaggcaaagagaagagtggtgcagagagaaaaaagagcagtgggaataggagctttgttccttgggttcttgggagcagcaggaagcactatgggcgcagcctcaatgacgctgacggtacaggccagacaattattgtctggtatagtgcagcagcagaacaatttgctgagggctattgaggcgcaacagcatctgttgcaactcacagtctggggcatcaagcagctccaggcaagaatcctggctgtggaaagatacctaaaggatcaacagctcctggggatttggggttgctctggaaaactcatttgcaccactgctgtgccttggaatgctagttggagtaataaatctctggaacagatttggaatcacacgacctggatggagtgggacagagaaattaacaattacacaagcttaatacactccttaattgaagaatcgcaaaaccagcaagaaaagaatgaacaagaattattggaattagataaatgggcaagtttgtggaattggtttaacataacaaattggctgtggtatataaaattattcataatgatagtaggaggcttggtaggtttaagaatagtttttgctgtactttctatagtgaatagagttaggcagggatattcaccattatcgtttcagacccacctcccaaccccgaggggacccgacaggcccgaaggaatagaagaagaaggtggagagagagacagagacagatccattcgattagtgaacggatctcgacggtatcggttaacttttaaaagaaaaggggggattggggggtacagtgcaggggaaagaatagtagacataatagcaacagacatacaaactaaagaattacaaaaacaaattacaaaaattcaaaattttatcgatcacgagactagcctcgagcgtggaggaaaaactgtttcatacagaaggcgtggaggaaaaactgtttcatacagaaggcgtggaggaaaaactgtttcatacagaaggcgtggaggaaaaactgtttcatacagaaggcgtggaggaaaaactgtttcatacagaaggcgtggaggaaaaactgtttcatacagaaggcgtctgcaggagactctagagggtatataatggtttaaacttaagcttggtaccgggcccccgaagacgcgtgccaccatggaacggatcgtgatctgcctgatggtcatcttcctgggcaccctggtgcacaagagcagctctcagggccaagaccggcacatgatccggatgagacagctgatcgacatcgtggaccagctgaagaactacgtgaacgacctggtgcctgagttcctgcctgctcctgaggacgtggaaacaaactgcgagtggagcgccttcagctgcttccagaaggcccagctgaaaagcgccaacaccggcaacaacgagcggatcatcaacgtgtccatcaagaagctgaagcggaagcctcctagcaccaacgccggaagaaggcagaagcacagactgacctgtcctagctgcgacagctacgagaagaagcctccaaaagagttcctggaacggttcaagagcctgctgcagaagatgatccaccagcacctgagcagcagaacccacggcagcgaggattcttgatgtacaagtaatcgaattcccacggggttggggttgcgccttttccaaggcagccctgggtttgcgcagggacgcggctgctctgggcgtggttccgggaaacgcagcggcgccgaccctgggtctcgcacattcttcacgtccgttcgcagcgtcacccggatcttcgccgctacccttgtgggccccccggcgacgcttcctgctccgcccctaagtcgggaaggttccttgcggttcgcggcgtgccggacgtgacaaacggaagccgcacgtctcactagtaccctcgcagacggacagcgccagggagcaatggcagcgcgccgaccgcgatgggctgtggccaatagcggctgctcagcggggcgcgccgagagcagcggccgggaaggggcggtgcgggaggcggggtgtggggcggtagtgtgggccctgttcctgcccgcgcggtgttccgcattctgcaagcctccggagcgcacgtcggcagtcggctccctcgttgaccgaatcaccgacctctctccccagggggatccaccggtcacgtggctagcgccaccnnnnnnnnnnnnnnnnnnnnnnnnnnnnnnnnnnnnnnnnnnnnnnnnnnnnnnnnnnnnnnnnnnnnnnnnnnnnnnnnnnnnnnnnnnnnnnnnnnnnnnnnnnnnnnnnnnnnnnnnnnnnnnnnnnnnnnnnnnnnnnnnnnnnnnnnnnnnnnnnnnnnnnnnnnnnnnnnnnnnnnnnnnnnnnnnnnnnnnnnnnnnnnnnnnnnnnnnnnnnnnnnnnnnnnnnnnnnnnnnnnnnnnnnnnnnnnnnnnnnnnnnnnnnnnnnnnnnnnnnnnnnnnnnnnnnnnnnnnnnnnnnnnnnnnnnnnnnnnnnnnnnnnnnnnnnnnnnnnnnnnnnnnnnnnnnnnnnnnnnnnnnnnnnnnnnnnnnnnnnnnnnnnnnnnnnnnnnnnnnnnnnnnnnnnnnnnnnnnnnnnnnnnnnnnnnnnnnnnnnnnnnnnnnnnnnnnnnnnnnnnnnnnnnnnnnnnnnnnnnnnnnnnnnnnnnnnnnnnnnnnnnnnnnnnnnnnnnnnnnnnnnnnnnnnnnnnnnnnnnnnnnnnnnnnnnnnnnnnnnnnnnnnnnnnnnnnnnnnnnnnnnnnnnnnnnnnnnnnnnnnnnnnnnnnnnnnnnnnnnnnnnnnnnnnnnnnnnnnnnnnnnnnnnnnnnnnnnnnnnnnnnnnnnnnnnnnnnnnnnnnnnnnnnnnnnnnnnnnnnnnnnnnnnnnnnnnnnnnnnnnnnnnnnnnnnnnnnnnnnnnnnnnnnnnnnnnnnnnnnnnnnnnnnnnnnnnnnnnnnnnnnnnnnnnnnnnnnnnnnnnnnnnnnnnnnnnnnnnnnnnnnnnnnnnnnnnnnnnnnnnnnnnnnnnnnnnnnnnnnnnnnnnnnnnnnnnnnnnnnnnnnnnnnnnnnnnnnnnnnnnnnnnnnnnnnnnnnnnnnnnnnnnnnnnnnnnnnnnnnnnnnnnnnnnnnnnnnnnnnnnnnnnnnnnnnnnnnnnnnnnnnnnnnnnnnnnnnnnnnnnnnnnnnnnnnnnnnnnnnnnnnnnnnnnnnnnnnnnnnnnnnnnnnnnnnnnnnnnnnnnnnnnnnnnnnnnnnnnnnnnnnnnnnnnnnnnnnnnnnnnnnnnnnnnnnnnnnnnnnnnnnnnnnnnnnnnnnnnnnnnnnnnnnnnnnnnnnnnnnnnnnnnnnnnnnnnnnnnnnnnnnnnnnnnnnnnnnnnnnnnnnnnnnnnnnnnnnnnnnnnnnnnnnnnnnnnnnnnnnnnnnnnnnnnnnnnnnnnnnnnnnnnnnnnnnnnnnnnnnnnnnnnnnnnnnnnnnnnnnnnnnnnnnnnnnnnnnnnnnnnnnnnnnnnnnnnnnnnnnnnnnnnnnnnnnnnnnnnnnnnnnnnnnnnnnnnnnnnnnnnnnnnnnnnnnnnnnnnnnnnnnnnnnnnnnnnnnnnnnnnnnnnnnnnnnnnnnnnnnnnnnnnnnnnnnnnntaggatccgccggcggccgcgtcgacaatcaacctctggattacaaaatttgtgaaagattgactggtattcttaactatgttgctccttttacgctatgtggatacgctgctttaatgcctttgtatcatgctattgcttcccgtatggctttcattttctcctccttgtataaatcctggttgctgtctctttatgaggagttgtggcccgttgtcaggcaacgtggcgtggtgtgcactgtgtttgctgacgcaacccccactggttggggcattgccaccacctgtcagctcctttccgggactttcgctttccccctccctattgccacggcggaactcatcgccgcctgccttgcccgctgctggacaggggctcggctgttgggcactgacaattccgtggtgttgtcggggaagctgacgtcctttccatggctgctcgcctgtgttgccacctggattctgcgcgggacgtccttctgctacgtcccttcggccctcaatccagcggaccttccttcccgcggcctgctgccggctctgcggcctcttccgcgtcttcgccttcgccctcagacgagtcggatctccctttgggccgcctccccgcctggaattcgagctcggtacctttaagaccaatgacttacaaggcagctgtagatcttagccactttttaaaagaaaaggggggactggaagggctaattcactcccaacgaagacaagatctgctttttgcttgtactgggtctctctggttagaccagatctgagcctgggagctctctggctaactagggaacccactgcttaagcctcaataaagcttgccttgagtgcttcaagtagtgtgtgcccgtctgttgtgtgactctggtaactagagatccctcagacccttttagtcagtgtggaaaatctctagcagtagtagttcatgtcatcttattattcagtatttataacttgcaaagaaatgaatatcagagagtgagaggaacttgtttattgcagcttataatggttacaaataaagcaatagcatcacaaatttcacaaataaagcatttttttcactgcattctagttgtggtttgtccaaactcatcaatgtatcttatcatgtctggctctagctatcccgcccctaactccgcccagttccgcccattctccgccccatggctgactaattttttttatttatgcagaggccgaggccgcctcggcctctgagctattccagaagtagtgaggaggcttttttggaggcctaggcttttgcgtcgagacgtacccaattcgccctatagtgagtcgtattacgcgcgctcactggccgtcgttttacaacgtcgtgactgggaaaaccctggcgttacccaacttaatcgccttgcagcacatccccctttcgccagctggcgtaatagcgaagaggcccgcaccgatcgcccttcccaacagttgcgcagcctgaatggcgaatggcgcgacgcgccctgtagcggcgcattaagcgcggcgggtgtggtggttacgcgcagcgtgaccgctacacttgccagcgccctagcgcccgctcctttcgctttcttcccttcctttctcgccacgttcgccggctttccccgtcaagctctaaatcgggggctccctttagggttccgatttagtgctttacggcacctcgaccccaaaaaacttgattagggtgatggttcacgtagtgggccatcgccctgatagacggtttttcgccctttgacgttggagtccacgttctttaatagtggactcttgttccaaactggaacaacactcaaccctatctcggtctattcttttgatttataagggattttgccgatttcggcctattggttaaaaaatgagctgatttaacaaaaatttaacgcgaattttaacaaaatattaacgtttacaatttcccaggtggcacttttcggggaaatgtgcgcggaacccctatttgtttatttttctaaatacattcaaatatgtatccgctcatgagacaataaccctgataaatgcttcaataatattgaaaaaggaagagtatgagtattcaacatttccgtgtcgcccttattcccttttttgcggcattttgccttcctgtttttgctcacccagaaacgctggtgaaagtaaaagatgctgaagatcagttgggtgcacgagtgggttacatcgaactggatctcaacagcggtaagatccttgagagttttcgccccgaagaacgttttccaatgatgagcacttttaaagttctgctatgtggcgcggtattatcccgtattgacgccgggcaagagcaactcggtcgccgcatacactattctcagaatgacttggttg

SEQ ID NO: 35 - DNA, 9692 bp, Artificial Sequence
  pCCL.PPT.NFATenhsyn.TRAIL.PGK.CAR.PRE
  enhancer 1858..2237: /note="CMV enhancer"
  promoter 2238..2441: /note="CMV promoter"
  LTR 2456..2636: /note="5´LTR, truncated"
  misc_signal 2683..2808: /note="psi packaging signal of HIV-1"
  misc_signal 3301..3534: /note="RRE of HIV-1"
  misc_signal 4030..4147: /note="cPPT/CTS"
  promoter 4174..4417: /note="NFATenhsyn"
  gene 4430..5275: /note="TRAIL"
  promoter 5299..5809: /note="hPGK promoter"
  gene 5842..7296: /note="placeholder for CAR"
  misc_signal 7323..7911: /note="WPRE"
  LTR 7998..8231: /note="3´LTR (delta U3)"
agtactcaccagtcacagaaaagcatcttacggatggcatgacagtaagagaattatgcagtgctgccataaccatgagtgataacactgcggccaacttacttctgacaacgatcggaggaccgaaggagctaaccgcttttttgcacaacatgggggatcatgtaactcgccttgatcgttgggaaccggagctgaatgaagccataccaaacgacgagcgtgacaccacgatgcctgtagcaatggcaacaacgttgcgcaaactattaactggcgaactacttactctagcttcccggcaacaattaatagactggatggaggcggataaagttgcaggaccacttctgcgctcggcccttccggctggctggtttattgctgataaatctggagccggtgagcgtgggtctcgcggtatcattgcagcactggggccagatggtaagccctcccgtatcgtagttatctacacgacggggagtcaggcaactatggatgaacgaaatagacagatcgctgagataggtgcctcactgattaagcattggtaactgtcagaccaagtttactcatatatactttagattgatttaaaacttcatttttaatttaaaaggatctaggtgaagatcctttttgataatctcatgaccaaaatcccttaacgtgagttttcgttccactgagcgtcagaccccgtagaaaagatcaaaggatcttcttgagatcctttttttctgcgcgtaatctgctgcttgcaaacaaaaaaaccaccgctaccagcggtggtttgtttgccggatcaagagctaccaactctttttccgaaggtaactggcttcagcagagcgcagataccaaatactgttcttctagtgtagccgtagttaggccaccacttcaagaactctgtagcaccgcctacatacctcgctctgctaatcctgttaccagtggctgctgccagtggcgataagtcgtgtcttaccgggttggactcaagacgatagttaccggataaggcgcagcggtcgggctgaacggggggttcgtgcacacagcccagcttggagcgaacgacctacaccgaactgagatacctacagcgtgagctatgagaaagcgccacgcttcccgaagggagaaaggcggacaggtatccggtaagcggcagggtcggaacaggagagcgcacgagggagcttccagggggaaacgcctggtatctttatagtcctgtcgggtttcgccacctctgacttgagcgtcgatttttgtgatgctcgtcaggggggcggagcctatggaaaaacgccagcaacgcggcctttttacggttcctggccttttgctggccttttgctcacatgttctttcctgcgttatcccctgattctgtggataaccgtattaccgcctttgagtgagctgataccgctcgccgcagccgaacgaccgagcgcagcgagtcagtgagcgaggaagcggaagagcgcccaatacgcaaaccgcctctccccgcgcgttggccgattcattaatgcagctggcacgacaggtttcccgactggaaagcgggcagtgagcgcaacgcaattaatgtgagttagctcactcattaggcaccccaggctttacactttatgcttccggctcgtatgttgtgtggaattgtgagcggataacaatttcacacaggaaacagctatgaccatgattacgccaagcgcgcaattaaccctcactaaagggaacaaaagctggagctgcaagcttggccattgcatacgttgtatccatatcataatatgtacatttatattggctcatgtccaacattaccgccatgttgacattgattattgactagttattaatagtaatcaattacggggtcattagttcatagcccatatatggagttccgcgttacataacttacggtaaatggcccgcctggctgaccgcccaacgacccccgcccattgacgtcaataatgacgtatgttcccatagtaacgccaatagggactttccattgacgtcaatgggtggagtatttacggtaaactgcccacttggcagtacatcaagtgtatcatatgccaagtacgccccctattgacgtcaatgacggtaaatggcccgcctggcattatgcccagtacatgaccttatgggactttcctacttggcagtacatctacgtattagtcatcgctattaccatggtgatgcggttttggcagtacatcaatgggcgtggatagcggtttgactcacggggatttccaagtctccaccccattgacgtcaatgggagtttgttttggcaccaaaatcaacgggactttccaaaatgtcgtaacaactccgccccattgacgcaaatgggcggtaggcgtgtacggtgggaggtctatataagcagagctcgtttagtgaaccggggtctctctggttagaccagatctgagcctgggagctctctggctaactagggaacccactgcttaagcctcaataaagcttgccttgagtgcttcaagtagtgtgtgcccgtctgttgtgtgactctggtaactagagatccctcagacccttttagtcagtgtggaaaatctctagcagtggcgcccgaacagggacttgaaagcgaaagggaaaccagaggagctctctcgacgcaggactcggcttgctgaagcgcgcacggcaagaggcgaggggcggcgactggtgagtacgccaaaaattttgactagcggaggctagaaggagagagatgggtgcgagagcgtcagtattaagcgggggagaattagatcgcgatgggaaaaaattcggttaaggccagggggaaagaaaaaatataaattaaaacatatagtatgggcaagcagggagctagaacgattcgcagttaatcctggcctgttagaaacatcagaaggctgtagacaaatactgggacagctacaaccatcccttcagacaggatcagaagaacttagatcattatataatacagtagcaaccctctattgtgtgcatcaaaggatagagataaaagacaccaaggaagctttagacaagatagaggaagagcaaaacaaaagtaagaccaccgcacagcaagcggccgctgatcttcagacctggaggaggagatatgagggacaattggagaagtgaattatataaatataaagtagtaaaaattgaaccattaggagtagcacccaccaaggcaaagagaagagtggtgcagagagaaaaaagagcagtgggaataggagctttgttccttgggttcttgggagcagcaggaagcactatgggcgcagcctcaatgacgctgacggtacaggccagacaattattgtctggtatagtgcagcagcagaacaatttgctgagggctattgaggcgcaacagcatctgttgcaactcacagtctggggcatcaagcagctccaggcaagaatcctggctgtggaaagatacctaaaggatcaacagctcctggggatttggggttgctctggaaaactcatttgcaccactgctgtgccttggaatgctagttggagtaataaatctctggaacagatttggaatcacacgacctggatggagtgggacagagaaattaacaattacacaagcttaatacactccttaattgaagaatcgcaaaaccagcaagaaaagaatgaacaagaattattggaattagataaatgggcaagtttgtggaattggtttaacataacaaattggctgtggtatataaaattattcataatgatagtaggaggcttggtaggtttaagaatagtttttgctgtactttctatagtgaatagagttaggcagggatattcaccattatcgtttcagacccacctcccaaccccgaggggacccgacaggcccgaaggaatagaagaagaaggtggagagagagacagagacagatccattcgattagtgaacggatctcgacggtatcggttaacttttaaaagaaaaggggggattggggggtacagtgcaggggaaagaatagtagacataatagcaacagacatacaaactaaagaattacaaaaacaaattacaaaaattcaaaattttatcgatcacgagactagcctcgagcgtggaggaaaaactgtttcatacagaaggcgtggaggaaaaactgtttcatacagaaggcgtggaggaaaaactgtttcatacagaaggcgtggaggaaaaactgtttcatacagaaggcgtggaggaaaaactgtttcatacagaaggcgtggaggaaaaactgtttcatacagaaggcgtctgcaggagactctagagggtatataatggtttaaacttaagcttggtaccgggcccccgaagacgcgtgccaccatggctatgatggaagtgcaaggcggacctagcctgggccagacatgtgtgctgatcgtgatcttcaccgtgctgctgcagagcctgtgtgtggccgtgacctacgtgtacttcaccaacgagctgaagcagatgcaggacaagtacagcaagagcggaatcgcctgcttcctgaaagaggacgacagctactgggaccccaacgacgaagagagcatgaacagcccctgctggcaagtgaagtggcagctgagacagctcgtgcggaagatgatcctgcggaccagcgaagagacaatcagcaccgtgcaagagaagcagcagaacatcagccctctcgtcagagagcggggacctcagagagtggccgctcacattactggcaccagaggcagaagcaacaccctgagcagccccaacagcaagaacgagaaggccctgggcagaaagatcaacagctgggagagcagcagatccggccacagctttctgagcaacctgcacctgagaaacggcgagctggtcatccacgagaagggcttctactacatctacagccagacctacttccggttccaagaggaaatcaaagagaataccaagaacgacaagcagatggtgcagtacatctataagtacacgagctaccccgatccgatcctgctgatgaagtccgccagaaacagctgctggtccaaggatgccgagtacggcctgtatagcatctaccaaggcggcatcttcgagctgaaagagaatgaccggatcttcgtgtccgtgaccaatgagcacctgatcgacatggaccacgaggccagctttttcggcgcctttcttgtgggctgatgtacaagtaatcgaattcccacggggttggggttgcgccttttccaaggcagccctgggtttgcgcagggacgcggctgctctgggcgtggttccgggaaacgcagcggcgccgaccctgggtctcgcacattcttcacgtccgttcgcagcgtcacccggatcttcgccgctacccttgtgggccccccggcgacgcttcctgctccgcccctaagtcgggaaggttccttgcggttcgcggcgtgccggacgtgacaaacggaagccgcacgtctcactagtaccctcgcagacggacagcgccagggagcaatggcagcgcgccgaccgcgatgggctgtggccaatagcggctgctcagcggggcgcgccgagagcagcggccgggaaggggcggtgcgggaggcggggtgtggggcggtagtgtgggccctgttcctgcccgcgcggtgttccgcattctgcaagcctccggagcgcacgtcggcagtcggctccctcgttgaccgaatcaccgacctctctccccagggggatccaccggtcacgtggctagcgccaccnnnnnnnnnnnnnnnnnnnnnnnnnnnnnnnnnnnnnnnnnnnnnnnnnnnnnnnnnnnnnnnnnnnnnnnnnnnnnnnnnnnnnnnnnnnnnnnnnnnnnnnnnnnnnnnnnnnnnnnnnnnnnnnnnnnnnnnnnnnnnnnnnnnnnnnnnnnnnnnnnnnnnnnnnnnnnnnnnnnnnnnnnnnnnnnnnnnnnnnnnnnnnnnnnnnnnnnnnnnnnnnnnnnnnnnnnnnnnnnnnnnnnnnnnnnnnnnnnnnnnnnnnnnnnnnnnnnnnnnnnnnnnnnnnnnnnnnnnnnnnnnnnnnnnnnnnnnnnnnnnnnnnnnnnnnnnnnnnnnnnnnnnnnnnnnnnnnnnnnnnnnnnnnnnnnnnnnnnnnnnnnnnnnnnnnnnnnnnnnnnnnnnnnnnnnnnnnnnnnnnnnnnnnnnnnnnnnnnnnnnnnnnnnnnnnnnnnnnnnnnnnnnnnnnnnnnnnnnnnnnnnnnnnnnnnnnnnnnnnnnnnnnnnnnnnnnnnnnnnnnnnnnnnnnnnnnnnnnnnnnnnnnnnnnnnnnnnnnnnnnnnnnnnnnnnnnnnnnnnnnnnnnnnnnnnnnnnnnnnnnnnnnnnnnnnnnnnnnnnnnnnnnnnnnnnnnnnnnnnnnnnnnnnnnnnnnnnnnnnnnnnnnnnnnnnnnnnnnnnnnnnnnnnnnnnnnnnnnnnnnnnnnnnnnnnnnnnnnnnnnnnnnnnnnnnnnnnnnnnnnnnnnnnnnnnnnnnnnnnnnnnnnnnnnnnnnnnnnnnnnnnnnnnnnnnnnnnnnnnnnnnnnnnnnnnnnnnnnnnnnnnnnnnnnnnnnnnnnnnnnnnnnnnnnnnnnnnnnnnnnnnnnnnnnnnnnnnnnnnnnnnnnnnnnnnnnnnnnnnnnnnnnnnnnnnnnnnnnnnnnnnnnnnnnnnnnnnnnnnnnnnnnnnnnnnnnnnnnnnnnnnnnnnnnnnnnnnnnnnnnnnnnnnnnnnnnnnnnnnnnnnnnnnnnnnnnnnnnnnnnnnnnnnnnnnnnnnnnnnnnnnnnnnnnnnnnnnnnnnnnnnnnnnnnnnnnnnnnnnnnnnnnnnnnnnnnnnnnnnnnnnnnnnnnnnnnnnnnnnnnnnnnnnnnnnnnnnnnnnnnnnnnnnnnnnnnnnnnnnnnnnnnnnnnnnnnnnnnnnnnnnnnnnnnnnnnnnnnnnnnnnnnnnnnnnnnnnnnnnnnnnnnnnnnnnnnnnnnnnnnnnnnnnnnnnnnnnnnnnnnnnnnnnnnnnnnnnnnnnnnnnnnnnnnnnnnnnnnnnnnnnnnnnnnnnnnnnnnnnnnnnnnnnnnnnnnnnnnnnnnnnnnnnnnnnnnnnnnnnnnnnnnnnnnnnnnnnnnnnnnnnnnnnnnnnnnnnnnnnnnnnnnnnnnnnnnnnnnnnnnnnnnnnnnnnnnnnnnnnnnnnnnnnnnnnnnnntaggatccgccggcggccgcgtcgacaatcaacctctggattacaaaatttgtgaaagattgactggtattcttaactatgttgctccttttacgctatgtggatacgctgctttaatgcctttgtatcatgctattgcttcccgtatggctttcattttctcctccttgtataaatcctggttgctgtctctttatgaggagttgtggcccgttgtcaggcaacgtggcgtggtgtgcactgtgtttgctgacgcaacccccactggttggggcattgccaccacctgtcagctcctttccgggactttcgctttccccctccctattgccacggcggaactcatcgccgcctgccttgcccgctgctggacaggggctcggctgttgggcactgacaattccgtggtgttgtcggggaagctgacgtcctttccatggctgctcgcctgtgttgccacctggattctgcgcgggacgtccttctgctacgtcccttcggccctcaatccagcggaccttccttcccgcggcctgctgccggctctgcggcctcttccgcgtcttcgccttcgccctcagacgagtcggatctccctttgggccgcctccccgcctggaattcgagctcggtacctttaagaccaatgacttacaaggcagctgtagatcttagccactttttaaaagaaaaggggggactggaagggctaattcactcccaacgaagacaagatctgctttttgcttgtactgggtctctctggttagaccagatctgagcctgggagctctctggctaactagggaacccactgcttaagcctcaataaagcttgccttgagtgcttcaagtagtgtgtgcccgtctgttgtgtgactctggtaactagagatccctcagacccttttagtcagtgtggaaaatctctagcagtagtagttcatgtcatcttattattcagtatttataacttgcaaagaaatgaatatcagagagtgagaggaacttgtttattgcagcttataatggttacaaataaagcaatagcatcacaaatttcacaaataaagcatttttttcactgcattctagttgtggtttgtccaaactcatcaatgtatcttatcatgtctggctctagctatcccgcccctaactccgcccagttccgcccattctccgccccatggctgactaattttttttatttatgcagaggccgaggccgcctcggcctctgagctattccagaagtagtgaggaggcttttttggaggcctaggcttttgcgtcgagacgtacccaattcgccctatagtgagtcgtattacgcgcgctcactggccgtcgttttacaacgtcgtgactgggaaaaccctggcgttacccaacttaatcgccttgcagcacatccccctttcgccagctggcgtaatagcgaagaggcccgcaccgatcgcccttcccaacagttgcgcagcctgaatggcgaatggcgcgacgcgccctgtagcggcgcattaagcgcggcgggtgtggtggttacgcgcagcgtgaccgctacacttgccagcgccctagcgcccgctcctttcgctttcttcccttcctttctcgccacgttcgccggctttccccgtcaagctctaaatcgggggctccctttagggttccgatttagtgctttacggcacctcgaccccaaaaaacttgattagggtgatggttcacgtagtgggccatcgccctgatagacggtttttcgccctttgacgttggagtccacgttctttaatagtggactcttgttccaaactggaacaacactcaaccctatctcggtctattcttttgatttataagggattttgccgatttcggcctattggttaaaaaatgagctgatttaacaaaaatttaacgcgaattttaacaaaatattaacgtttacaatttcccaggtggcacttttcggggaaatgtgcgcggaacccctatttgtttatttttctaaatacattcaaatatgtatccgctcatgagacaataaccctgataaatgcttcaataatattgaaaaaggaagagtatgagtattcaacatttccgtgtcgcccttattcccttttttgcggcattttgccttcctgtttttgctcacccagaaacgctggtgaaagtaaaagatgctgaagatcagttgggtgcacgagtgggttacatcgaactggatctcaacagcggtaagatccttgagagttttcgccccgaagaacgttttccaatgatgagcacttttaaagttctgctatgtggcgcggtattatcccgtattgacgccgggcaagagcaactcggtcgccgcatacactattctcagaatgacttggttg